European Patent Specification EP 3 789 042 B1, published November 6, 2024. Title: METHOD FOR PRODUCING ANTI-HER3 ANTIBODY-DRUG CONJUGATE. Applicant: Daiichi Sankyo Company, Limited. The sequence listing filed with the application follows.

SEQUENCE LISTING (584 sequences)

SEQ ID NO: 1 - DNA, 342 bp, Artificial
  Antibody
gaggtgcagctggtggagtctggaggaggcttgatccagcctggggggtccctgagactctcctgtgcagcctctgggttcaccgtcagtagcaactacatgagctgggtccgccaggctccagggaaggggctggattgggtctcagttatttatagcggtggtagcacatactacgcagactccgtgaagggccgattcaccatctccagagacaattccaagaacacgctgtatcttcaaatgaacagcctgagagccgaggacacggccgtgtattactgtgcgagagggcagtggctggacgtctggggccaagggaccacggtcaccgtctcctca

SEQ ID NO: 2 - protein, 114 aa, Artificial
  Antibody
EVQLVESGGGLIQPGGSLRLSCAASGFTVSSNYMSWVRQAPGKGLDWVSVIYSGGSTYYADSVKGRFTISRDNSKNTLYLQMNSLRAEDTAVYYCARGQWLDVWGQGTTVTVSS

SEQ ID NO: 3 - DNA, 336 bp, Artificial
  Antibody
gatattgtgatgactcagtctccactctccctgcccgtcacccctggagagccggcctccatctcctgcaggtcaagtcagagcctcctgcatagtaatggatacaactatttggattggtacctgcagaggccagggcagtctccacaactcctgttctatttgggttttcatcgggcctccggggtccctgacaggttcagtggcagtggatcaggcacagattttacactgaaaatcagcagagtggaggctgaggatgttggggtttattactgcaggcaagctctacaaactccgctcactttcggcggagggaccaaggtggagatcaaa

SEQ ID NO: 4 - protein, 112 aa, Artificial
  Antibody
DIVMTQSPLSLPVTPGEPASISCRSSQSLLHSNGYNYLDWYLQRPGQSPQLLFYLGFHRASGVPDRFSGSGSGTDFTLKISRVEAEDVGVYYCRQALQTPLTFGGGTKVEIK

SEQ ID NO: 5 - DNA, 374 bp, Artificial
  Antibody
caggtgcagctgcaggagtcgggcccaggactggtgaagccttcacagaccctgtccctcacctgtactgtctctggtggctccatcagcagtggtggttactactggagctggatccgccagcacccagggaagggcctggagtggattgggtacatctattccagtgggagcacctactacaacccgtccctcaagagtcgagttaccatatcagtagacacgtctaagaaccagttctccctgaagctgagctctgtgactgccgcggacacggccgtgtattactgtgcgagagatagggaactggaactttactactactactacggtatggacgtctggggccaagggaccacggtcaccgtctcctc

SEQ ID NO: 6 - protein, 124 aa, Artificial
  Antibody
QVQLQESGPGLVKPSQTLSLTCTVSGGSISSGGYYWSWIRQHPGKGLEWIGYIYSSGSTYYNPSLKSRVTISVDTSKNQFSLKLSSVTAADTAVYYCARDRELELYYYYYGMDVWGQGTTVTVS

SEQ ID NO: 7 - DNA, 336 bp, Artificial
  Antibody
gatattgtgatgactcagtctccactctccctgcccgtcacccctggagagccggcctccatctcctgcaggtctagtcagagcctcctgtatagtaatggatacaactatttggattggtacctgcagaagccagggcagtctccacagctcctgatctatttgggttctaatcgggcctccggggtccctgacaggttcagtggcagtggatcaggcacagattttacactgaaaatcagcagagtggaggctgaggatgttgggatttattactgcatgcaagctctacaaactccgctcactttcggcggagggaccaaggtggagatcaaa

SEQ ID NO: 8 - protein, 112 aa, Artificial
  Antibody
DIVMTQSPLSLPVTPGEPASISCRSSQSLLYSNGYNYLDWYLQKPGQSPQLLIYLGSNRASGVPDRFSGSGSGTDFTLKISRVEAEDVGIYYCMQALQTPLTFGGGTKVEIK

SEQ ID NO: 9 - DNA, 357 bp, Artificial
  Antibody
cagatcaccttgaaggagtctggtcctacgctggtgaaacccacacagaccctcacgctgacctgcaccttctctgggttctcactcagcactagtggagtgggtgtgggctggatccgtcagcccccaggaaaggccctggactggcttgcactcatttattggaatgatgataagcgctacagcccatctctgaagagcaggctcaccatcaccaaggacacctccaaaaaccaggtggtccttacaatgaccaacatggatcttgtggacacagccacatattactgtgtacacagagacgaagttcgagggtttgactactggggccagggaaccctggtcaccgtctcctca

SEQ ID NO: 10 - protein, 119 aa, Artificial
  Antibody
QITLKESGPTLVKPTQTLTLTCTFSGFSLSTSGVGVGWIRQPPGKALDWLALIYWNDDKRYSPSLKSRLTITKDTSKNQVVLTMTNMDLVDTATYYCVHRDEVRGFDYWGQGTLVTVSS

SEQ ID NO: 11 - DNA, 336 bp, Artificial
  Antibody
gatgttgtgatgactcagtctccactctccctgcccgtcacccttggacagccggcctccatctcctgcaggtctagtcaaagcctcgtatacagtgatggatacacctacttgcattggtttcagcagaggccaggccaatctccaaggcgccttatttataaggtttctaactgggactctggggtcccagacagattcagcggcagtgggtcaggcactgatttcacactgaaaatcagcagggtggaggctgaggatgttggggtttattactgcatgcaaggtgcacactggccgatcaccttcggccaagggacacgactggagattaaa

SEQ ID NO: 12 - protein, 112 aa, Artificial
  Antibody
DVVMTQSPLSLPVTLGQPASISCRSSQSLVYSDGYTYLHWFQQRPGQSPRRLIYKVSNWDSGVPDRFSGSGSGTDFTLKISRVEAEDVGVYYCMQGAHWPITFGQGTRLEIK

SEQ ID NO: 13 - DNA, 374 bp, Artificial
  Antibody
caggtgcagctgcaggagtcgggcccaggactggtgaagccttcacagaccctgtccctcacctgcactgtctctggtggctccatcagcagtggtgggtactactggagctggatccgccagcacccagggaagggcctggagtggattgggtacatctattacagtgggagcacctactacaacccgtccctcaagagtcgagttaccatatcagtagacacgtctaagaaccagttctccctgaagctgagctctgtgactgccgcggacacggccgtgtatttctgtgcgagagatcgggaacttgagggttactccaactactacggtgtggacgtctggggccaagggaccacggtcaccgtctcctc

SEQ ID NO: 14 - protein, 124 aa, Artificial
  Antibody
QVQLQESGPGLVKPSQTLSLTCTVSGGSISSGGYYWSWIRQHPGKGLEWIGYIYYSGSTYYNPSLKSRVTISVDTSKNQFSLKLSSVTAADTAVYFCARDRELEGYSNYYGVDVWGQGTTVTVS

SEQ ID NO: 15 - DNA, 321 bp, Artificial
  Antibody
gacatccagatgacccagtctccatcctccctgtctgcatctgtaggagacagagtcaccatcacttgccgggcaagtcaggccattagcaactatttaaattggtatcagcagaaaccagggaaagcccctaagctcctgatctatgctgcatccagtttgcaaagtggggtcccatcaaggttcagtggcagtggatctgggacagatttcactctcaccatcagcagcctgcagcctgaagattttgcaacttattactgtcaacagaataatagtctcccgatcaccttcggccaagggacacgactggagattaaa

SEQ ID NO: 16 - protein, 107 aa, Artificial
  Antibody
DIQMTQSPSSLSASVGDRVTITCRASQAISNYLNWYQQKPGKAPKLLIYAASSLQSGVPSRFSGSGSGTDFTLTISSLQPEDFATYYCQQNNSLPITFGQGTRLEIK

SEQ ID NO: 17 - DNA, 354 bp, Artificial
  Antibody
gaggtgcagctggtgcagtctggagcagaggtgaaaaagcccggggagtctctgaagatctcctgtaagggttctggatacagctttaccagctactggatcggctgggtgcgccagatgcccgggaaaggcctggagtggatggggatcatctatcctggtgactctgataccagatacagcccgtccttccaaggccaggtcaccatctcagccgacaagtccatcagcaccgcctacctgcagtggagcagcctgaaggcctcggacaccgccatgtattactgtgcgagacatgaaaactacggtgactacaactactggggccagggaaccctggtcaccgtctcctca

SEQ ID NO: 18 - protein, 118 aa, Artificial
  Antibody
EVQLVQSGAEVKKPGESLKISCKGSGYSFTSYWIGWVRQMPGKGLEWMGIIYPGDSDTRYSPSFQGQVTISADKSISTAYLQWSSLKASDTAMYYCARHENYGDYNYWGQGTLVTVSS

SEQ ID NO: 19 - DNA, 321 bp, Artificial
  Antibody
gacatccagatgacccagtctccatcctccctgtctgcatctgtcggagacagagtcaccatcacttgccgggcaagtcagagcattcgcagctatttaaattggtatcagcagaaaccagggaaagcccctaagctcctgatctatgctgcttccagtttgcaaagtggggtcccatcaaggttcagtggcagtggatctgggacagatttcactctcaccatcagcagtctgcaacctgaagattttgcactttactgctgtcaacagagtaacggttccccgctcactttcggcggagggaccaaggtggagatcaaa

SEQ ID NO: 20 - protein, 107 aa, Artificial
  Antibody
DIQMTQSPSSLSASVGDRVTITCRASQSIRSYLNWYQQKPGKAPKLLIYAASSLQSGVPSRFSGSGSGTDFTLTISSLQPEDFALYCCQQSNGSPLTFGGGTKVEIK

SEQ ID NO: 21 - DNA, 380 bp, Artificial
  Antibody
caggtgcagctgcaggagtcgggcccaggactggtgaagccttcacagaccctgtccctcacctgcactgtctctggtggctccatcagcagtggtggttactactggagctggatccgccagcacccagggaagggcctggagtggattgggtacatctattacagtgggagcacctactacaacccgtccctcaggagtcgagttaccatatcagtagacacgtctaagaaccagttctccctgaagctgagctctgtgactgccgcggacacggccgtgtattactgtgcgagagatagagagagagagtgggatgattacggtgacccccaaggtatggacgtctggggccaagggaccacggtcaccgtctcctc

SEQ ID NO: 22 - protein, 126 aa, Artificial
  Antibody
QVQLQESGPGLVKPSQTLSLTCTVSGGSISSGGYYWSWIRQHPGKGLEWIGYIYYSGSTYYNPSLRSRVTISVDTSKNQFSLKLSSVTAADTAVYYCARDREREWDDYGDPQGMDVWGQGTTVTVS

SEQ ID NO: 23 - DNA, 321 bp, Artificial
  Antibody
gacatccagatgacccagtctccatcctccctgtctgcatctgtaggagacagagtcaccatcacttgccgggcaagtcagagcattagcagctatttacattggtatcagcagaaaccagggaaagcccctaagctcctgatccatgctgcatccagtttacaaagtggggtcccatcaaggttcagtggcagtggatctgggacagatttcactctcaccatcagtagtctgcaacctgaagattttgcaacttactactgtcaacagagttacagtaacccgctcactttcggcggagggaccaaggtggagatccaa

SEQ ID NO: 24 - protein, 107 aa, Artificial
  Antibody
DIQMTQSPSSLSASVGDRVTITCRASQSISSYLHWYQQKPGKAPKLLIHAASSLQSGVPSRFSGSGSGTDFTLTISSLQPEDFATYYCQQSYSNPLTFGGGTKVEIQ

SEQ ID NO: 25 - DNA, 354 bp, Artificial
  Antibody
gaggtgcagctggtgcagtctggagcagaggtgaaaaagcccggggagtctctgaagatctcctgtaagggttctggatacagctttaccagctactggatcggctgggtgcgccagatgcccgggaaaggcctggagtggatggggatcatctggcctggtgactctgataccatatacagcccgtccttccaaggccaggtcaccatctcagccgacaagtccatcagcaccgcctacctgcagtggagcagcctgaaggcctcggacaccgccatgtattactgtgcgagacatgaaaactacggtgactacaactactggggccagggaaccctggtcaccgtctcctca

SEQ ID NO: 26 - protein, 118 aa, Artificial
  Antibody
EVQLVQSGAEVKKPGESLKISCKGSGYSFTSYWIGWVRQMPGKGLEWMGIIWPGDSDTIYSPSFQGQVTISADKSISTAYLQWSSLKASDTAMYYCARHENYGDYNYWGQGTLVTVSS

SEQ ID NO: 27 - DNA, 321 bp, Artificial
  Antibody
gacatccagatgacccagtctccatcctccctgtctgcatctgtgggagacagagtcaccatcacttgccgggcaagtcagagcattcgaagttatttaaattggtatcagcagaaaccggggaatgcccctaaactcctgatctatgctgcatccagtttgcaaagtggggtcccatcaaggttcagtggcagtggatctgggacagatttcactctcaccatcagcagtctgcaacctgaagattttgcactttactactgtcaacagagtatcagttccccgctcactttcggcggagggaccaaggtggagatcaaa

SEQ ID NO: 28 - protein, 107 aa, Artificial
  Antibody
DIQMTQSPSSLSASVGDRVTITCRASQSIRSYLNWYQQKPGNAPKLLIYAASSLQSGVPSRFSGSGSGTDFTLTISSLQPEDFALYYCQQSISSPLTFGGGTKVEIK

SEQ ID NO: 29 - DNA, 374 bp, Artificial
  Antibody
caggtgcagctggtgcagtctggggctgaggtgaagaagcctggggcctcagtgaaggtctcctgcaaggcttctggatacaccttcaccagttatgatatcaactgggtgcgacaggccactggacaagggcttgagtggatgggatggatgaaccctaacagtggtgacactggctatgcacaggtgttccagggcagagtcaccatgacctggaacacctccataagcacagcctacatggaactgagcagcctgagatctgaggacacggccgtgtattactgtgcgagatttggggatctcccgtatgactacagttactacgaatggttcgacccctggggccagggaaccctggtcaccgtctcctc

SEQ ID NO: 30 - protein, 124 aa, Artificial
  Antibody
QVQLVQSGAEVKKPGASVKVSCKASGYTFTSYDINWVRQATGQGLEWMGWMNPNSGDTGYAQVFQGRVTMTWNTSISTAYMELSSLRSEDTAVYYCARFGDLPYDYSYYEWFDPWGQGTLVTVS

SEQ ID NO: 31 - DNA, 321 bp, Artificial
  Antibody
gacatccagatgacccagtctccatcctccctgtctgcatctgtaggagacagagtcaccatcacttgccgggcaagccagagcattagcagctatttaaattggtatcagcagagaccagggaaagcccctaagctcctgatctatgcagcatccagtttgcaaagtggggtcccatcaaggttcagtggcagtggatctgggacagatttcactctcaccatcagcagtctgcaacctgaagattttgcaacttactactgtcaacagagttacagtaccccgctcactttcggcggagggaccaaggtggagatcaaa

SEQ ID NO: 32 - protein, 107 aa, Artificial
  Antibody
DIQMTQSPSSLSASVGDRVTITCRASQSISSYLNWYQQRPGKAPKLLIYAASSLQSGVPSRFSGSGSGTDFTLTISSLQPEDFATYYCQQSYSTPLTFGGGTKVEIK

SEQ ID NO: 33 - DNA, 386 bp, Artificial
  Antibody
caggtacagctgcagcagtcaggtccaggactggtgaagccctcgcagaccctctcactcacctgtgccatctccggggacagtgtctctagcaacagtgctgcttggaactggatcaggcagtccccatcgagaggccttgagtggctgggaaggacatactacaggtccaagtggtataatgattatgcagtatctgtgaaaagtcgaataaccatcaacccagacacatccaagaaccagttctccctgcagctgaactctgtgactcccgaggacacggctgtgtattactgtgcaagagatctctacgatttttggagtggttatccctactactacggtatggacgtctggggccaagggaccacggtcaccgtctcctc

SEQ ID NO: 34 - protein, 128 aa, Artificial
  Antibody
QVQLQQSGPGLVKPSQTLSLTCAISGDSVSSNSAAWNWIRQSPSRGLEWLGRTYYRSKWYNDYAVSVKSRITINPDTSKNQFSLQLNSVTPEDTAVYYCARDLYDFWSGYPYYYGMDVWGQGTTVTVS

SEQ ID NO: 35 - DNA, 383 bp, Artificial
  Antibody
caggtacagctgcagcagtcaggtccaggactggtgaagccctcgcagaccctctcactcacctgtgccatctccggggacagtgtctctagcaacagtgctgcttggaactggatcaggcagtccccatcgagaggccttgagtggctgggaaggacatactacaggtccaagtggtataatgattatgcagtatctgtgaaaagtcgaataaccatcaacccagacacatccaagaaccagttctccctgcagctgaactctgtgactcccgaggacacggctgtgtattactgtgcaagagattactatggttcggggagtttctactactactacggtatggacgtctggggccaagggaccacggtcaccgtctcctc

SEQ ID NO: 36 - protein, 127 aa, Artificial
  Antibody
QVQLQQSGPGLVKPSQTLSLTCAISGDSVSSNSAAWNWIRQSPSRGLEWLGRTYYRSKWYNDYAVSVKSRITINPDTSKNQFSLQLNSVTPEDTAVYYCARDYYGSGSFYYYYGMDVWGQGTTVTVS

SEQ ID NO: 37 - DNA, 321 bp, Artificial
  Antibody
gacatccagatgacccagtctccatcctccctgtctgcatctgtaggagacagagtcaccatcacttgccgggcaagtcagagcattagcagctatttaaattggtatcagcagaaaccagggaaagcccctaaggtcctgatctatgctgcatccaatttgcaaagtggggtcccatcaaggttcagtggcagtggatctgggacagatttcactctcaccatcagcagtctgcaacctgaagattttgcaacttactactgtcaacagagttacagtacccctcggacgttcggccaagggaccaaggtggaaatcaaa

SEQ ID NO: 38 - protein, 107 aa, Artificial
  Antibody
DIQMTQSPSSLSASVGDRVTITCRASQSISSYLNWYQQKPGKAPKVLIYAASNLQSGVPSRFSGSGSGTDFTLTISSLQPEDFATYYCQQSYSTPRTFGQGTKVEIK

SEQ ID NO: 39 - DNA, 371 bp, Artificial
  Antibody
caggtgcagctgcaggagtcgggcccaggactggtgaagccttcggagaccctgtccctcacctgcactgtctctggtggctccatcagtagttactactggagctggatccggcagcccgccgggaagggactggagtggattgggcatatctataccagtgggagcaccaactacaacccctccctcaagagtcgagtcaccatgtcagtagacacgtccaagaaccagttctccctgaagctgagctctgtgaccgccgcggacacggccgtgtattactgtgcgagagaagcgatttttggagtgggcccctactactactacggtatggacgtctggggccaagggaccacggtcaccgtctcctc

SEQ ID NO: 40 - protein, 123 aa, Artificial
  Antibody
QVQLQESGPGLVKPSETLSLTCTVSGGSISSYYWSWIRQPAGKGLEWIGHIYTSGSTNYNPSLKSRVTMSVDTSKNQFSLKLSSVTAADTAVYYCAREAIFGVGPYYYYGMDVWGQGTTVTVS

SEQ ID NO: 41 - DNA, 377 bp, Artificial
  Antibody
caggtgcagctggtgcagtctggggctgaggtgaagaagcctggggcctcagtgaaggtctcctgcaaggcttctggatacaccttcaccggctactatatgcactgggtgcgacaggcccctggacaagggcttgagtggatgggatggatcaaccctaatattggtggcacaaactgtgcacagaagtttcagggcagggtcaccatgaccagggacacgtccatcagcacagcctacatggagctgagcaggctgagatctgacgacacggccgtgtattactgtgcgagagggggacggtatagcagcagctggtcctactactactacggtatggacgtctggggccaagggaccacggtcaccgtctcctc

SEQ ID NO: 42 - protein, 125 aa, Artificial
  Antibody
QVQLVQSGAEVKKPGASVKVSCKASGYTFTGYYMHWVRQAPGQGLEWMGWINPNIGGTNCAQKFQGRVTMTRDTSISTAYMELSRLRSDDTAVYYCARGGRYSSSWSYYYYGMDVWGQGTTVTVS

SEQ ID NO: 43 - DNA, 336 bp, Artificial
  Antibody
gatattctgatgacccagactccactctctctgtccgtcacccctggacagccggcctccatctcctgcaagtctagtcagagcctcctgcttagtgatggagggacctatttgtattggtacctgcagaagccaggccagcctccacagctcctgatctatgaagtttccaaccggttctctggagtgccagataggttcagtggcagcgggtcagggacagatttcacactgaaaatcagccgggtggaggctgaggatgttggggtttattactgcatgcaaagtatgcagcttccgatcaccttcggccaagggacacgactggaaattaaa

SEQ ID NO: 44 - protein, 112 aa, Artificial
  Antibody
DILMTQTPLSLSVTPGQPASISCKSSQSLLLSDGGTYLYWYLQKPGQPPQLLIYEVSNRFSGVPDRFSGSGSGTDFTLKISRVEAEDVGVYYCMQSMQLPITFGQGTRLEIK

SEQ ID NO: 45 - DNA, 380 bp, Artificial
  Antibody
caggtgcagctgcaggagtcgggcccaggactggtgaagccttcggagaccctgtccctcacctgcactgtctctggtggctccgtcagcagtggtggttactactggagctggatccggcagcccccagggaagggactggagtggattgggtatatctattacagtgggagcaccaactacaacccctccctcaagagtcgagtcaccatatcagtagacacgtccaagaaccagttctccctgaagctgagctctgtgaccgctgcggacacggccgtgtattactgtgcgagagggggggacagtaactacgaggattactactactactacggtatggacgtctggggccaagggaccacggtcaccgtctcctc

SEQ ID NO: 46 - protein, 126 aa, Artificial
  Antibody
QVQLQESGPGLVKPSETLSLTCTVSGGSVSSGGYYWSWIRQPPGKGLEWIGYIYYSGSTNYNPSLKSRVTISVDTSKNQFSLKLSSVTAADTAVYYCARGGDSNYEDYYYYYGMDVWGQGTTVTVS

SEQ ID NO: 47 - DNA, 321 bp, Artificial
  Antibody
gacatccagatgacccagtctccatcctccctgtctgcatctgtaggagacagagtcaccatcacttgccgggcaagtcagagcattagcatctatttacattggtatcagcagaaaccagggaaagcccctaagctcttgatctctgctgcatccagtttgcaaagtggggtcccgtcaaggttcagtggcagtggatctgggacagatttcactctcaccatcagaagtctgcaacctgaagattttgcaacttactactgtcaacagagttacacttccccgatcaccttcggccaagggacacgactggagattaaa

SEQ ID NO: 48 - protein, 107 aa, Artificial
  Antibody
DIQMTQSPSSLSASVGDRVTITCRASQSISIYLHWYQQKPGKAPKLLISAASSLQSGVPSRFSGSGSGTDFTLTIRSLQPEDFATYYCQQSYTSPITFGQGTRLEIK

SEQ ID NO: 49 - DNA, 380 bp, Artificial
  Antibody
caggtgcagctgcaggagtcgggcccaggactggtgaagccttcggagaccctgtccctcacctgcactgtctctggtggctccatcagtagttactactggagctggatccggcagcccccagggaagggactggagtggattgggtatatctattacagtgggagcaccaactacaacccctccctcaagagtcgagtcaccatatcagtagacacgtccaagcaccagttctccctgaagctgagctctgtgaccgctgcggacacggccgtgtattactgtgcgagagattcgagttactatgatagtagtggttattacttatactactacgctatggacgtctggggccaagggaccacggtcaccgtctcctc

SEQ ID NO: 50 - protein, 126 aa, Artificial
  Antibody
QVQLQESGPGLVKPSETLSLTCTVSGGSISSYYWSWIRQPPGKGLEWIGYIYYSGSTNYNPSLKSRVTISVDTSKHQFSLKLSSVTAADTAVYYCARDSSYYDSSGYYLYYYAMDVWGQGTTVTVS

SEQ ID NO: 51 - DNA, 339 bp, Artificial
  Antibody
gacatcgtgatgacccagtctccagactccctggctgtgtctctgggcgagagggccaccatcaactgcaagtccagccagagtgttttatacagctccaacaataagaactacttagcttggtaccagcagaaaccaggacagcctcctaagctgctcatttcctgggcatctacccgggaatccggggtccctgaccgattcagtggcagcgggtctgggacagatttcactctcaccatcagcagcctgcaggctgaagatgtggcagtttattactgtcagcaatattatactactcctctcactttcggccctgggaccaaagtggatatcaaa

SEQ ID NO: 52 - protein, 113 aa, Artificial
  Antibody
DIVMTQSPDSLAVSLGERATINCKSSQSVLYSSNNKNYLAWYQQKPGQPPKLLISWASTRESGVPDRFSGSGSGTDFTLTISSLQAEDVAVYYCQQYYTTPLTFGPGTKVDIK

SEQ ID NO: 53 - DNA, 357 bp, Artificial
  Antibody
gaggtgcaactggtggagtctgggggaggcttggtacagcctggggggtccctgagactctcctgtgcagcctctggattcaccttcagtatctatagcatgaactgggtccgccaggctccagggaaggggctggagtgggtttcatacattagtagtagtagtagtaccatatactacgcagactctgtgaagggccgattcaccatctccagagacaatgccaagaactcactgtatctgcaaatgaacagcctgagagacgaggacacggctgtgtattactgtgcgagagataggggtgacttcgatgcttttgatatctggggccaagggacaatggtcaccgtctcttca

SEQ ID NO: 54 - protein, 119 aa, Artificial
  Antibody
EVQLVESGGGLVQPGGSLRLSCAASGFTFSIYSMNWVRQAPGKGLEWVSYISSSSSTIYYADSVKGRFTISRDNAKNSLYLQMNSLRDEDTAVYYCARDRGDFDAFDIWGQGTMVTVSS

SEQ ID NO: 55 - DNA, 321 bp, Artificial
  Antibody
gacatccagatgacccagtctccatcctccctgtctgcatctgtaggagacagagtcaccatcacttgccaggcgagtcaggacattaccaactatttgaattggtatcagcagaaaccagggaaagcccctaagctcctgatctacgatgcatccaatttggaaacaggggtcccatcaaggttcagtggaagtggatctgggacagattttactttcaccatcagcagcctgcagcctgaagatattgcaacatataactgtcaacagtgtgaaaatttcccgatcaccttcggccaagggacacgactggagattaaa

SEQ ID NO: 56 - protein, 107 aa, Artificial
  Antibody
DIQMTQSPSSLSASVGDRVTITCQASQDITNYLNWYQQKPGKAPKLLIYDASNLETGVPSRFSGSGSGTDFTFTISSLQPEDIATYNCQQCENFPITFGQGTRLEIK

SEQ ID NO: 57 - DNA, 336 bp, Artificial
  Antibody
gatattgtgatgactcagtctccactctccctgcccgtcacccctggagagccggcctccatctcctgcaggtctagtcagagcctcctgtatagtaatggatacaagtatttggattggtacctgcagaagccagggcagtctccacagctcctgatctatttgggttctaatcgggcctccggggtccctgacaggttcagtggcagtggatcaggcacagattttacactgaaaatcagcagagtggaggctgaggatgttggggtttattattgcatgcaggctctacaaactccgatcaccttcggccaagggacacgactggagattaaa

SEQ ID NO: 58 - protein, 112 aa, Artificial
  Antibody
DIVMTQSPLSLPVTPGEPASISCRSSQSLLYSNGYKYLDWYLQKPGQSPQLLIYLGSNRASGVPDRFSGSGSGTDFTLKISRVEAEDVGVYYCMQALQTPITFGQGTRLEIK

SEQ ID NO: 59 - DNA, 374 bp, Artificial
  Antibody
caggtgcagctgcaggagtcgggcccaggactggtgaagccttcggagaccctgtccctcacctgcactgtctctggtggctccgtcagcagtggtggttactactggaactggatccggcagcccccagggaagggactggagtggattgggtatatcaattacagtgggagcaccaactacaacccctccctcaagagtcgagtcaccatatcagtagacacgtccaagaaccagttctccctgaagctgagctctgtgaccgctgcggacacggccgtgtattactgtgcgagagatcgagaactggaactttactactactactacggtatggacgtctggggccaagggaccacggtcaccgtctcctc

SEQ ID NO: 60 - protein, 124 aa, Artificial
  Antibody
QVQLQESGPGLVKPSETLSLTCTVSGGSVSSGGYYWNWIRQPPGKGLEWIGYINYSGSTNYNPSLKSRVTISVDTSKNQFSLKLSSVTAADTAVYYCARDRELELYYYYYGMDVWGQGTTVTVS

SEQ ID NO: 61 - DNA, 374 bp, Artificial
  Antibody
caggtgcagctgcaggagtcgggcccaggactggtgaagccttctgagaccctgtccctcacctgcactgtctctggtggctccgtcagcagtggtggttactactggaactggatccggcagcccccagggaagggactggagtggattgggtatatcaattacagtgggagcaccaactacaacccctccctcaagagtcgagtcaccatatcagtagacacgtccaagaaccagttctccctgaagctgagctctgtgaccgctgcggacacggccgtgtattactgtgcgagagatcgagaactggaactttactactactactacggtatggacgtctggggccaagggaccacggtcaccgtctcctc

SEQ ID NO: 62 - protein, 124 aa, Artificial; identical to SEQ ID NO: 60
  Antibody

SEQ ID NO: 63 - DNA, 336 bp, Artificial
  Antibody
gatattgtgatgactcagtctccactctccctgcccgtcacccctggagagccggcctccatctcctgcaggtctagtcagagcctcctgtatagtaatggatacaagtatttggattggtacctgcagaagccagggcagtctccacagctcatgatctatttgggttctaatcgggcctccggggtccctgacaggttcagtggcagtggatcaggcacagattttacactgaaaatcagcagagtggaggctgaggatgttggggtttattattgcatgcaggctctacaaactccgatcaccttcggccaagggacacgactggagattaaa

SEQ ID NO: 64 - protein, 112 aa, Artificial
  Antibody
DIVMTQSPLSLPVTPGEPASISCRSSQSLLYSNGYKYLDWYLQKPGQSPQLMIYLGSNRASGVPDRFSGSGSGTDFTLKISRVEAEDVGVYYCMQALQTPITFGQGTRLEIK

SEQ ID NO: 65 - DNA, 363 bp, Artificial
  Antibody
caggtgcagctggtggagtctgggggaggcgtggtccagcctgggaggtccctgagactctcctgtgcagcgtctggattcaccttcagtagctatggcatgcactgggtccgccaggctccaggcaaggggctggagtgggtggcagttatatggtatgatggaagtaataaatactatgcagactccgtgaagggccgattcaccatctccagagacaattccaagaacacgctgtatctgcaaatgaacagcctgagagccgaggacacggctgtgtattactgtgcgagagcagctcgccttgactactactacggtatggacgtctggggccaagggaccacggtcaccgtctcctca

SEQ ID NO: 66 - protein, 121 aa, Artificial
  Antibody
QVQLVESGGGVVQPGRSLRLSCAASGFTFSSYGMHWVRQAPGKGLEWVAVIWYDGSNKYYADSVKGRFTISRDNSKNTLYLQMNSLRAEDTAVYYCARAARLDYYYGMDVWGQGTTVTVSS

SEQ ID NO: 67 - DNA, 321 bp, Artificial
  Antibody
gacatccagatgacccagtctccatcctccctgtctgcatctgtaggagacagagtctccatcacttgccgggcaagtcagagcattaacagctatttaaattggtttcagcagaagccagggaaagcccctcagctcctgatctttggtgcatccggtttgcaaagtggggtcccatcaaggttcagtggcagtggatctgggacagatttcactctcaccatcaacagtctgcaacctgaagattttgcaacttactactgtcaacagagttacagttccccgctcaccttcggccaagggacacgactggagattaaa

SEQ ID NO: 68 - protein, 107 aa, Artificial
  Antibody
DIQMTQSPSSLSASVGDRVSITCRASQSINSYLNWFQQKPGKAPQLLIFGASGLQSGVPSRFSGSGSGTDFTLTINSLQPEDFATYYCQQSYSSPLTFGQGTRLEIK

SEQ ID NO: 69 - DNA, 351 bp, Artificial
  Antibody
caggtgcagctacagcagtggggcgcaggactgttgaagccttcggagaccctgtccctcacctgcgctgtctatggtgggtccttcagtggttactactggagctggatccgccagcccccagggaaggggctggagtggattggggaaatcaatcatagtggaagcaccaactacaacccgtccctcaagagtcgagtcaccatatcagtagaaacgtccaagaaccagttctccctgaagctgagctctgtgaccgccgcggacacggctgtgtattactgtgcgagagataagtggacctggtacttcgatctctggggccgtggcaccctggtcactgtctcctca

SEQ ID NO: 70 - protein, 117 aa, Artificial [sequence omitted]

SEQ ID NO: 71 - DNA, 339 bp, Artificial
  Antibody
gacatcgagatgacccagtctccagactccctggctgtgtctctgggcgagagggccaccatcaactgcaggtccagccagagtgttttatacagctccagcaataggaactacttagcttggtaccagcagaacccaggacagcctcctaagctgctcatttactgggcttctacccgggaatccggggtccctgaccgattcagtggcagcgggtctgggacagatttcactctcaccatcagcagcctgcaggctgaagatgtggcagtttattactgtcagcaatattatagtactcctcggacgttcggccaagggaccaaggtggaaatcaaa

SEQ ID NO: 72 - protein, 113 aa, Artificial [sequence omitted]

SEQ ID NO: 73 - DNA, 374 bp, Artificial
  Antibody
caggtgcagctgcaggagtcgggcccaggactggtgaagccttcacagaccctgtccctcacctgcactgtctctggtggctccatcagcagtggtggttactactggagctggatccgccagcacccagggaagggcctggagtggatggggaacatctattacagtgggagcacctactacaacccgtccctcaagagtcgagttaccatatcagtagacacgtctgagaaccagttctccctgaagctgaactctgtgactgccgcggacacggccgtatattactgtgcgagagggggaactggaaccaattactactactactacggtatggacgtctggggccaagggaccacggtcaccgtctcctc

SEQ ID NO: 74 - protein, 124 aa, Artificial
  Antibody
QVQLQESGPGLVKPSQTLSLTCTVSGGSISSGGYYWSWIRQHPGKGLEWMGNIYYSGSTYYNPSLKSRVTISVDTSENQFSLKLNSVTAADTAVYYCARGGTGTNYYYYYGMDVWGQGTTVTVS

SEQ ID NO: 75 - DNA, 324 bp, Artificial
  Antibody
gaaattgtgttgacgcagtctccaggcaccctgtctttgtctccaggggaaagagccaccctctcctgcagggccagtcagagtgttagcagcagctacttagcctggtaccagcagaaacctggccaggctcccaggctcctcatctatggtgcatccagctgggccactggcatcccaaacaggttcagtggcagtgggtctgggacagacttcactctcaccatcagcagactggagcctgaagattttgcagtgtattactgtcagcagtatggtagctcaccgctcactttcggcggagggaccaaggtggagatcaaa

SEQ ID NO: 76 - protein, 108 aa, Artificial
  Antibody
EIVLTQSPGTLSLSPGERATLSCRASQSVSSSYLAWYQQKPGQAPRLLIYGASSWATGIPNRFSGSGSGTDFTLTISRLEPEDFAVYYCQQYGSSPLTFGGGTKVEIK

SEQ ID NO: 77 - DNA, 377 bp, Artificial
  Antibody
caggtgcagctgcaggagtcgggcccaggactggtgaagccttcacagaccctgtccctcacctgcactgtctctggtgtctccatcagcagtggtggttactactggagctggatccgccagcacccagggatgggcctggagtggattgggtacatctattacagtgggagcacctactacaacccgtccctcaagagtcgagtcaccatatcagaagacacgtctaagaaccagttctccctgaagctgagctctgtgactgccgcggacacggccgtgtattactgtgcgagagattccgagtccgagtatagcagctcgtcgaactacggtatggacgtctggggccaagggaccacggtcaccgtctcctc

SEQ ID NO: 78 - protein, 125 aa, Artificial
  Antibody
QVQLQESGPGLVKPSQTLSLTCTVSGVSISSGGYYWSWIRQHPGMGLEWIGYIYYSGSTYYNPSLKSRVTISEDTSKNQFSLKLSSVTAADTAVYYCARDSESEYSSSSNYGMDVWGQGTTVTVS

SEQ ID NO: 79 - DNA, 377 bp, Artificial; identical to SEQ ID NO: 77
  Antibody

SEQ ID NO: 80 - protein, 125 aa, Artificial; identical to SEQ ID NO: 78
  Antibody

SEQ ID NO: 81 - DNA, 321 bp, Artificial
  Antibody
gacatccagatgacccagtctccatcctccctgtctgcatctgtaggagacagaatcaccatcacttgccgggcaagtcagaccattagcagctatttaaattggtatcagcagaaaccagggaaagcccctaagctcctgatctatgctgcatccagtttgcaaggtggggtcccatcaaggttcagtggcagtgtatctgggacagatttcaccctcaccgtcagcagtctgcaacctgaagattttgcaacttactactgtcaacagagttacagtaacccgctcactttcggcggagggaccaaggtggagatcaaa

SEQ ID NO: 82 - protein, 107 aa, Artificial
  Antibody
DIQMTQSPSSLSASVGDRITITCRASQTISSYLNWYQQKPGKAPKLLIYAASSLQGGVPSRFSGSVSGTDFTLTVSSLQPEDFATYYCQQSYSNPLTFGGGTKVEIK

SEQ ID NO: 83 - DNA, 371 bp, Artificial
  Antibody
gaggtgcagctggtgcagtctggagcagaggtgaaaaagcccggggagtctctgaagatctcctgtaagggttctggatacagttttaccagctactggatcggctgggtgcgccagatgcccgggaaaggcctggagtggatggggatcatctatcctggtgactctgataccagatacagcccgtccttccaaggccaggtcaccatgtcagccgacaagtccatcagtaccgcctacctgcagctgagcagccatgaaggcctcggacaccgccatgtattactgtgcgagacagatggctggaaactacgtacatcacgggtgatcgagacgtcctggggccaagggaccacggtcaccgtctcctc

SEQ ID NO: 84 - protein, 123 aa, Artificial
  Antibody
EVQLVQSGAEVKKPGESLKISCKGSGYSFTSYWIGWVRQMPGKGLEWMGIIYPGDSDTRYSPSFQGQVTMSADKSISTAYLQLSSHEGLGHRHVLLCETDGWKLRTSRVIETSWGQGTTVTVS

SEQ ID NO: 85 - DNA, 324 bp, Artificial
  Antibody
gaaattgtgttgacgcagtctccaggcaccctgtctttgtctccaggggaaagagccaccctctcctgcagggccagtcagagtgttatcagcatctacttagcctggtaccagcagaaacctggccaggctcccaggctcctcatctatggtgcatccagcagggccactggcatcccagacaggttcagtggcagtgggtctgggacagacttcactctcaccatcagcagactggagcctgaagattttgcagtgtattactgtcagcagtatggtagctcaccgtgcagttttggccaggggaccaaactggagatcaaa

SEQ ID NO: 86 - protein, 108 aa, Artificial
  Antibody
EIVLTQSPGTLSLSPGERATLSCRASQSVISIYLAWYQQKPGQAPRLLIYGASSRATGIPDRFSGSGSGTDFTLTISRLEPEDFAVYYCQQYGSSPCSFGQGTKLEIK

SEQ ID NO: 87 - DNA, 366 bp, Artificial
  Antibody
caggtgcagctgcaggagtcgggcccaggactggtgaagccttcacagaccctgtccctcacctgcactgtctctggtggctccatcagcagtggtgattactactggagctggatccgccagcacccagggaagggcctggagtggattgggtacatctattacagtgggagcacctactacaacccgtccctcaggagtcgagttaccatatcagtagacacgtctaagaaccagttctccctgaagctgagctctgtgactgccgcggacacggccgtgtattactgtgcgagagcggattacgatttttggagtggttattttgactactggggccagggaaccctggtcaccgtctcctca

SEQ ID NO: 88 - protein, 122 aa, Artificial
  Antibody
QVQLQESGPGLVKPSQTLSLTCTVSGGSISSGDYYWSWIRQHPGKGLEWIGYIYYSGSTYYNPSLRSRVTISVDTSKNQFSLKLSSVTAADTAVYYCARADYDFWSGYFDYWGQGTLVTVSS

SEQ ID NO: 89 - DNA, 322 bp, Artificial
  Antibody
gacatccagatgacccagtctccatcctccctgtctgcatctgtaggagacagagtcaccatcacttgccgggcaagtcagggcattagaaatgatttaggctggtatcagcagatacctgggaaagcccctaagcgcctgatctatgctgcatccagtttgcaaagtggggtcccatcaaggttcagcggcagtggatctgggacagaattcactctcacaatcaacagcctgcagcctgaagattttgcaacttattactgtctacagcataatggttacccgtggacgttcggccaagggaccaaggtggaaatcaaac

SEQ ID NO: 90 - protein, 107 aa, Artificial
  Antibody
DIQMTQSPSSLSASVGDRVTITCRASQGIRNDLGWYQQIPGKAPKRLIYAASSLQSGVPSRFSGSGSGTEFTLTINSLQPEDFATYYCLQHNGYPWTFGQGTKVEIK

SEQ ID NO: 91 - DNA, 366 bp, Artificial
  Antibody
caggtgcagctgcaggagtcgggcccaggactggtgaagccttcacagaccctgtccctcacctgcactgtctctggtggctccatcagcagtggtgattactactggagctggatccgccagcacccagggaagggcctggagtggattggatacatctattacagtgggagcacctactacaacccgtccctcaagagtcgagttaccatatcagtagacacgtctaagaaccagttctccctgaagctgagctctgtgactgccgcggacacggccgtgtattactgtgcgagagcggattacgatttttggagtggttattttgactactggggccagggaaccctggtcaccgtctcctca

SEQ ID NO: 92 - protein, 122 aa, Artificial
  Antibody
QVQLQESGPGLVKPSQTLSLTCTVSGGSISSGDYYWSWIRQHPGKGLEWIGYIYYSGSTYYNPSLKSRVTISVDTSKNQFSLKLSSVTAADTAVYYCARADYDFWSGYFDYWGQGTLVTVSS

SEQ ID NO: 93 - DNA, 322 bp, Artificial
  Antibody
gacttccagatgacccagtctccatcctccctgtctgcatctgtaggagacagagtcaccatcacttgccgggcaagtcaggacattcgaaatgatttaggctggtatcggcagaaacctgggaaagcccctaagcgcctgatctatgctgcatccagtttgcaaagtggggtcccatcaaggttcagcggcagtggatctgggacagaattcactctcacaatcagcagcctgcagcctgaagattttgcaacttattactgtctacagcataatagttacccgtggacgttcggccaagggaccaaggtggaaatcaaac

SEQ ID NO: 94 - protein, 107 aa, Artificial
  Antibody
DFQMTQSPSSLSASVGDRVTITCRASQDIRNDLGWYRQKPGKAPKRLIYAASSLQSGVPSRFSGSGSGTEFTLTISSLQPEDFATYYCLQHNSYPWTFGQGTKVEIK

SEQ ID NO: 95 - DNA, 366 bp, Artificial
  Antibody
caggtgcagctgcaggagtcgggcccaggactggtgaagccttcacagaccctgtccctcacctgcactgtctctggtggctccatcagcagtggtgattactactggagctggatccgccagcacccagggaagggcctggagtggattggatacatctattacagtgggagcacctactacaacccgtccctcaagagtcgagttaccatatcaatagacacgtctaagaaccagttctccctgaagctgagctctgtgactgccgcggacacggccgtgtattactgtgcgagagcggattacgatttttggaatggttattttgactactggggccagggaaccctggtcaccgtctcctca

SEQ ID NO: 96 - protein, 122 aa, Artificial
  Antibody
QVQLQESGPGLVKPSQTLSLTCTVSGGSISSGDYYWSWIRQHPGKGLEWIGYIYYSGSTYYNPSLKSRVTISIDTSKNQFSLKLSSVTAADTAVYYCARADYDFWNGYFDYWGQGTLVTVSS

SEQ ID NO: 97 - DNA, 321 bp, Artificial
  Antibody
gacatccagatgacccagtctccatcctccctgtctgcatctgtaggagacagagtcaccatcacttgccgggcaagtcaggacattagaaatgatttaggctggtatcggcagaaacctgggaaagcccctaagcgcctgatctatgctgcatccagtttgcaaagtggggtcccatcaaggttcagcggcagtggatctgggacagaattcactctcacaatcagcagcctgcagcctgaagattttgcaacttattactgtctacagcataatagttacccgtggacgttcggccaagggaccaaggtggaaatcaaa

SEQ ID NO: 98 - protein, 107 aa, Artificial
  Antibody
DIQMTQSPSSLSASVGDRVTITCRASQDIRNDLGWYRQKPGKAPKRLIYAASSLQSGVPSRFSGSGSGTEFTLTISSLQPEDFATYYCLQHNSYPWTFGQGTKVEIK

SEQ ID NO: 99 - DNA, 366 bp, Artificial
  Antibody
caggtgcagctgcaggagtcgggcccaggactggtgaagcctacacagaccctgtccctcacctgcactgtctctggtggctccatcagcagtggtgattactactggagctggatccgccagcacccagggaagggcctggagtggattgggtacatctattacagtgggagcacctactacaacccgtccctcaagagtcgacttaccatatcagtagacacgtctaagaaccagttctccctgaagctgagctctgtgactgccgcggacacggccgtgtattactgtgcgagagcagattacgatttttggagtggttactttgactactggggccagggaaccctggtcaccgtctcctca

SEQ ID NO: 100 - protein, 122 aa, Artificial
  Antibody
QVQLQESGPGLVKPTQTLSLTCTVSGGSISSGDYYWSWIRQHPGKGLEWIGYIYYSGSTYYNPSLKSRLTISVDTSKNQFSLKLSSVTAADTAVYYCARADYDFWSGYFDYWGQGTLVTVSS

SEQ ID NO: 101 - DNA, 321 bp, Artificial
  Antibody
gacatccagatgacccagtctccatcctccctgtctgcatctgtaggagacagagtcaccatcacttgccgggcaagtcagggcattagaaatgatttaggctggtatcagcagaaaccagggaaagcccctaagcgcctgatctatgctgcatccagtttgcaaagtggggtcccatcaaggttcagcggcagtggatctgggacagaattcactctcacaatcagcagcctgcagcctgaagattttgcaacttattactgtctacagcataataattacccgtggacgttcggccaagggaccaaggtggaaatcaaa

SEQ ID NO: 102 - protein, 107 aa, Artificial
  Antibody
DIQMTQSPSSLSASVGDRVTITCRASQGIRNDLGWYQQKPGKAPKRLIYAASSLQSGVPSRFSGSGSGTEFTLTISSLQPEDFATYYCLQHNNYPWTFGQGTKVEIK

SEQ ID NO: 103 - DNA, 366 bp, Artificial
  Antibody
caggtgcagctgcaggagtcgggcccaggactggtgaagccttcacagaccctgtccctcacctgcactgtctctggtggctccatcagtagtggtgattactactggagctggatccgccagcacccagggaagggcctggagtggattgggtacatctattacagtgggagcacctactacaacccgtccctcaagagtcgagttaccatatcagtagacacgtctaagaaccagttctccctgaagttgagctctgtgactgccgcggacacggccgtgtattactgtgcgagagccgattacgatttttggagtggttattttgactactggggccagggaaccctggtcaccgtctcctca

SEQ ID NO: 104 - protein, 122 aa, Artificial; identical to SEQ ID NO: 92
  Antibody

SEQ ID NO: 105 - DNA, 321 bp, Artificial; identical to SEQ ID NO: 101
  Antibody

SEQ ID NO: 106 - protein, 107 aa, Artificial; identical to SEQ ID NO: 102
  Antibody

SEQ ID NO: 107 - DNA, 351 bp, Artificial
  Antibody
caggtgcagctgcaggagtcgggcccaggactggtgaagccttcacagaccctgtccctcacctgcactgtctctggtggctccatcagcagtggtggttactactggagctggatccgccagcacccagggaagggcctggagtggattgggtacatctattacagtgggagcacctactacaacccgtccctcaagagtcgagttaccatatcagtagacacgtctaagaaccagttctccctgaagctgagctctgtgactgccgcggacacggccgtgtattactgtgcgagagaggacgacggtatggacgtctggggccaagggaccacggtcaccgtctcctca

SEQ ID NO: 108 - protein, 117 aa, Artificial
  Antibody
QVQLQESGPGLVKPSQTLSLTCTVSGGSISSGGYYWSWIRQHPGKGLEWIGYIYYSGSTYYNPSLKSRVTISVDTSKNQFSLKLSSVTAADTAVYYCAREDDGMDVWGQGTTVTVSS

SEQ ID NO: 109 - DNA, 336 bp, Artificial
  Antibody
gatattgtgatgactcagtctccactctccctgcccgtcacccctggagagccggcctccatttcctgcaggtctagtcagagcctcctgcatagtaatggatacaactatttggaatggtacctgcagaagccagggcagtccccacagttcatgatttatttggggtctaatcgggcctccggggtccctgacaggttcagtggcagtggatcaggcacagattttacactgaaaatcagcagagtggaggctgaggatgttggggtttattactgcatgcaagctctacaaactccgatcaccttcggccaagggacacgactggagattaaa

SEQ ID NO: 110 - protein, 112 aa, Artificial
  Antibody
DIVMTQSPLSLPVTPGEPASISCRSSQSLLHSNGYNYLEWYLQKPGQSPQFMIYLGSNRASGVPDRFSGSGSGTDFTLKISRVEAEDVGVYYCMQALQTPITFGQGTRLEIK

SEQ ID NO: 111 - DNA, 366 bp, Artificial
  Antibody
caggtgcagctgcaggagtcgggcccaggactggtgaagccttcacagaccctgtccctcacctgcactgtctctggtggctccatcagcagtggtgattactactggagctggatccgccagtacccagggaagggcctggagtggattgggtacatctattacagtgggagcacctactacaacccgtccctcaagagtcgagttaccatatcagtagacacgtctaagaaccagttctccctgaagctgaggtctgtgactgccgcggacacggccgtgtattactgtgcgagagcggattacgatttttggagtggttattttgactactggggccagggaaccctggtcaccgtctcctca

SEQ ID NO: 112 - protein, 122 aa, Artificial
  Antibody
QVQLQESGPGLVKPSQTLSLTCTVSGGSISSGDYYWSWIRQYPGKGLEWIGYIYYSGSTYYNPSLKSRVTISVDTSKNQFSLKLRSVTAADTAVYYCARADYDFWSGYFDYWGQGTLVTVSS

SEQ ID NO: 113 - DNA, 322 bp, Artificial
  Antibody
gacatccagatgacccagtctccatcctccctgtctgcatctgtaggagacagagtcaccatcacttgccgggcaagtcagggcattagaaatgatttaggctggtatcagcagaaaccagggaaagcccctaagcgcctgatctatgctgcatccagtttgcaaagtggggtcccatcaaggttcagcggcagtggatctgggacagaattcactctcacaatcagcagcctgcagcctgaagattttgcaacttattactgtctacagcataatacttacccgtggacgttcggccaagggaccaaggtggaaatcaaac

SEQ ID NO: 114 - protein, 107 aa, Artificial
  Antibody
DIQMTQSPSSLSASVGDRVTITCRASQGIRNDLGWYQQKPGKAPKRLIYAASSLQSGVPSRFSGSGSGTEFTLTISSLQPEDFATYYCLQHNTYPWTFGQGTKVEIK

SEQ ID NO: 115 - DNA, 372 bp, Artificial
  Antibody
caggtgcagctgcaggagtcgggcccaggactggtgaagccttcggagaccctgtccctcacctgcactgtctctggtggctccgtcagcagtggtggttactactggagctggatccggcagcccccagggaagggactggagtggattgggtatatctattacagtgggagcaccaactacaacccctccctcaagagtcgagtcaccatatcagtagacacgtccaagaaccagttctccctgaagctgagctctgtgaccgctgcggacacggccgtgtattactgtgcgagagatggggacgtggatacagctatggtcgatgcttttgatatctggggccaagggacaatggtcaccgtctcctca

SEQ ID NO: 116 - protein, 124 aa, Artificial
  Antibody
QVQLQESGPGLVKPSETLSLTCTVSGGSVSSGGYYWSWIRQPPGKGLEWIGYIYYSGSTNYNPSLKSRVTISVDTSKNQFSLKLSSVTAADTAVYYCARDGDVDTAMVDAFDIWGQGTMVTVSS

SEQ ID NO: 117 - DNA, 324 bp, Artificial
  Antibody
gaaattgtattgacgcagtctccaggcaccctgtctttgtctccaggggaaagagccaccctctcctgcagggccagtcagagtttaagcggcaactacttagcctggtaccagcagaagcctggccaggctcccaggctcatcatctgtggtgcatccagcagggccactggcatcccagacaggttcagtggcagtgggtctgggacagacttcactctcaccatcacaagactggagcctgaagattttgcagtgtattactgtcagcagtatgataggtcaccgctcactttcggcggagggaccaaggtggagatcaaa

SEQ ID NO: 118 - protein, 108 aa, Artificial
  Antibody
EIVLTQSPGTLSLSPGERATLSCRASQSLSGNYLAWYQQKPGQAPRLIICGASSRATGIPDRFSGSGSGTDFTLTITRLEPEDFAVYYCQQYDRSPLTFGGGTKVEIK

SEQ ID NO: 119 - DNA, 366 bp, Artificial
  Antibody
caggtgcagctgcaggagtcgggcccaggactggtgaagccttcacagaccctgtccctcacctgcactgtctctggtggctccatcagcagtggtgattactactggagctggatccgccagcacccagggaagggcctggagtggattgggtacatctattacagtgggagcacctactacaacccgtccctcaagagtcgagttaccatatcagtagacacgtctaagaaccagttctccctgaagctgagctctgtgactgccgcggacacggccgtgtattactgtgcgagaggagattacgatttttggagtggagagtttgactactggggccagggaaccctggtcaccgtctcctca

SEQ ID NO: 120 - protein, 122 aa, Artificial
  Antibody
QVQLQESGPGLVKPSQTLSLTCTVSGGSISSGDYYWSWIRQHPGKGLEWIGYIYYSGSTYYNPSLKSRVTISVDTSKNQFSLKLSSVTAADTAVYYCARGDYDFWSGEFDYWGQGTLVTVSS

SEQ ID NO: 121 - DNA, 386 bp, Artificial
  Antibody
caggtgcagctgcaggagtcgggcccaggactggtgaagccttcacagaccctgtccctcacctgcactgtctctggtggctccatcagcagtggtggttactactggagctggatccgccagcacccagggaagggcctggagtggattgggtacatctatgacagtgggagcacctactacaacccgtccctcaagagtcgagttaccatatcagtagacacgtctaagaaccagttctccctgaagctgaggtctgtgactgccgcggacacggccgtgtattactgtgcgagagatcaggggcaggacggatacagctatggttacggctactactacggtatggacgtctggggccaagggaccacggtcaccgtctcctc

SEQ ID NO: 122 - protein, 128 aa, Artificial
  Antibody
QVQLQESGPGLVKPSQTLSLTCTVSGGSISSGGYYWSWIRQHPGKGLEWIGYIYDSGSTYYNPSLKSRVTISVDTSKNQFSLKLRSVTAADTAVYYCARDQGQDGYSYGYGYYYGMDVWGQGTTVTVS

SEQ ID NO: 123 - DNA, 321 bp, Artificial
  Antibody
gacatccagatgacccagtctccatcctccctgtctgcatctgtaggagacagagtcaccatcacttgccaggcgagtcaggacattagcaattatttaaattggtatcagcagaaaccagggaaagcccctaaactcctgatctacgttgcatccaatttggaaacaggggtcccatcaaggttcagtggaagtggatctgggacagattttactttcaccatcagcagcctgcagcctgaagatattgcaacatattactgtcaacagtgtgataatctccctctcactttcggcggagggaccaaggtggagatcaaa

SEQ ID NO: 124 - protein, 107 aa, Artificial
  Antibody
DIQMTQSPSSLSASVGDRVTITCQASQDISNYLNWYQQKPGKAPKLLIYVASNLETGVPSRFSGSGSGTDFTFTISSLQPEDIATYYCQQCDNLPLTFGGGTKVEIK

SEQ ID NO: 125 - DNA, 365 bp, Artificial
  Antibody
caggtgcagctgcaggagtcgggcccaggactggtgaagccttcacagaccctgtccctcacctgcactgtctctggtggctccatcagcagtggtgattactactggagctggatccgccagcacccagggaagggcctggagtggattggatacatctattacagtgggagcacctactacaacccgtccctcaagagtcgagttaccatatcagtagacacgtctaagaaccagttctccctgaagctgagctctgtgactgccgcggacacggccgtgtattactgtgcgagagcggattacgatttttggagtggttattttgactactggggccagggaaccctggtcaccgtctcctc

SEQ ID NO: 126 - protein, 121 aa, Artificial
  Antibody
QVQLQESGPGLVKPSQTLSLTCTVSGGSISSGDYYWSWIRQHPGKGLEWIGYIYYSGSTYYNPSLKSRVTISVDTSKNQFSLKLSSVTAADTAVYYCARADYDFWSGYFDYWGQGTLVTVS

SEQ ID NO: 127 - DNA, 322 bp, Artificial
  Antibody
gacatccagatgacccagtctccatcctccctgtctgcatctgtaggagacagagtcaccatcacttgccgggcaagtcaggacattagaaatgatttaggctggtatcggcagaaacctgggaaagcccctaagcgcctgatctatgctgcatcccgtttgcaaagtggggtcccatcaaggttcagcggcagtggatctgggacagaattcactctcacaatcagcagcctgcagcctgaagattttgcaacttattactgtctacagcataatagttacccgtggacgttcggccaagggaccaaggtggaaatcaaac

SEQ ID NO: 128 - protein, 107 aa, Artificial
  Antibody
DIQMTQSPSSLSASVGDRVTITCRASQDIRNDLGWYRQKPGKAPKRLIYAASRLQSGVPSRFSGSGSGTEFTLTISSLQPEDFATYYCLQHNSYPWTFGQGTKVEIK

SEQ ID NO: 129 - DNA, 366 bp, Artificial
  Antibody
caggtgcagctgcaggagtcgggcccaggactggtgaagccttcacagaccctgtccctcacctgcactgtctctggtggctccatcagcagtggtgattactactggagctggatccgccagcacccagggaagggcctggagtggattgggtacatctattacagtgggagcacctactacaacccgtccctcaagagtcgagttaccatatcagtagacacgtctaagaaccagttctccctgaagctgagctctgtgactgccgcggacacggccgtgtattactgtgcgagagccgattacgatttttggagtggttattttgactactggggccagggaaccctggtcaccgtctcctca

SEQ ID NO: 130 - protein, 122 aa, Artificial; identical to SEQ ID NO: 92
  Antibody

SEQ ID NO: 131 - DNA, 322 bp, Artificial
  Antibody
gacatccagatgacccagtctccatcctccctgtctgcatctgtaggagacagagtcaccatcacttgccgggcaagtcagggcattagaaatgatttaggctggtatcagcagaaaccagggaaagcccctaagcgcctgatctatgctgcatccagtttgcaaaatggggtcccatcaaggttcagcggcagtggatctgggacagaattcactctcacaatcagcagcctgcagcctgaagattttgcaacttattactgtctacagcataatagttacccgtggacgttcggccaagggaccaaggtggaaatcaaac

SEQ ID NO: 132 - protein, 107 aa, Artificial
  Antibody
DIQMTQSPSSLSASVGDRVTITCRASQGIRNDLGWYQQKPGKAPKRLIYAASSLQNGVPSRFSGSGSGTEFTLTISSLQPEDFATYYCLQHNSYPWTFGQGTKVEIK

SEQ ID NO: 133 - DNA, 365 bp, Artificial
  Antibody
caggtgcagctgcaggagtcgggcccaggactggtgaagccttcacagaccctgtccctcacctgcactgtctctggtggctccatcagcagtggtgattactactggagctggatccgccagcacccagggaagggcctggagtggattgggtacatctattacagtgggagcacctactacaacccgtccctcaagagtcgagttaccatatcagtagacacgtctaagaaccagttctccctgaagctgagctctgtgactgccgcggacacggccgtgtattactgtgcgagagcggattacgatttttggagtggttattttgactactggggccagggaatcctggtcaccgtctcctc

SEQ ID NO: 134 - protein, 121 aa, Artificial
  Antibody
QVQLQESGPGLVKPSQTLSLTCTVSGGSISSGDYYWSWIRQHPGKGLEWIGYIYYSGSTYYNPSLKSRVTISVDTSKNQFSLKLSSVTAADTAVYYCARADYDFWSGYFDYWGQGILVTVS

SEQ ID NO: 135 - DNA, 322 bp, Artificial
  Antibody
gacatccagatgacccagtctccatcctccctgtctgcatctgtaggagacagagtcaccatcacttgccgggcaagtcagggcattagaaatgatttaggctggtatcagcagaaaccagggaaagcccctaagcgcctgatttatgctgcatccagtttgcaaagtggggtcccatcaaggttcagcggcagtggatctgggacagaattcactctcacaatcagcagcctgcagcctgaagattttgcaacttattactgtctacagcataatagttacccgtggacgttcggccaagggaccaaggtggaaatcaaac

SEQ ID NO: 136 - protein, 107 aa, Artificial
  Antibody
DIQMTQSPSSLSASVGDRVTITCRASQGIRNDLGWYQQKPGKAPKRLIYAASSLQSGVPSRFSGSGSGTEFTLTISSLQPEDFATYYCLQHNSYPWTFGQGTKVEIK

SEQ ID NO: 137 - DNA, 366 bp, Artificial
  Antibody
caggtgcagctgcaggagtcgggcccaggactggtgaagccttcacagaccctgtccctcacctgcactgtctctggtggctccatcagtagtggtgattactactggagctggatccgccagcacccagggaagggcctggagtggattgggtacatctattacagtgggagcacctactacaacccgtccctcaagagtcgagttaccatatcagtagacacgtctaagaaccagttctccctgaagttgagctctgtgactgccgcggacacggccgtgtattactgtgcgagagccgattacgatttttggaatggttattttgactactggggccagggaaccctggtcaccgtctcctca

SEQ ID NO: 138 - protein, 122 aa, Artificial
  Antibody
QVQLQESGPGLVKPSQTLSLTCTVSGGSISSGDYYWSWIRQHPGKGLEWIGYIYYSGSTYYNPSLKSRVTISVDTSKNQFSLKLSSVTAADTAVYYCARADYDFWNGYFDYWGQGTLVTVSS

SEQ ID NO: 139 - DNA, 321 bp, Artificial; identical to SEQ ID NO: 101
  Antibody

SEQ ID NO: 140 - protein, 107 aa, Artificial; identical to SEQ ID NO: 102
  Antibody

SEQ ID NO: 141 - DNA, 366 bp, Artificial; identical to SEQ ID NO: 129
  Antibody

SEQ ID NO: 142 - protein, 122 aa, Artificial; identical to SEQ ID NO: 92
  Antibody

SEQ ID NO: 143 - DNA, 322 bp, Artificial
  Antibody
gacatccagctgacccagtctccatcctccctgtctgcatctgtaggagacagagtcaccatcacttgccgggcaagtcagggcattagaaatgatttaggctggtatcagcagaaaccagggaaagcccctaagcgcctgatctatgctgcatccagtttgcaaaatggggtcccatcaaggttcagcggcagtggatctgggacagaattcactctcacaatcagcagcctgcagcctgaagattttgcaacttattactgtctacagcataatagttacccgtggacgttcggccaagggaccaaggtggaaatcaaac

SEQ ID NO: 144 - protein, 107 aa, Artificial
  Antibody
DIQLTQSPSSLSASVGDRVTITCRASQGIRNDLGWYQQKPGKAPKRLIYAASSLQNGVPSRFSGSGSGTEFTLTISSLQPEDFATYYCLQHNSYPWTFGQGTKVEIK

SEQ ID NO: 145 - DNA, 365 bp, Artificial
  Antibody
caggtgcagctgcaggagtcgggcccaggactggtgaagccttcacagaccctgtccctcacctgcactgtctctggtggctccatcagcagtggtgattactactggagctggatccgccagtacccagggaagggcctggagtggattgggtacatctattacagtgggagcacctactacaacccgtccctcaagagtcgagttaccatatcagtagacacgtctaagaaccagttctccctgaagctgggctctgtgactgccgcggacacggccgtgtatttctgtgcgagagccgattacgatttttggagtggttattttgacttctggggccagggaaccctggtcaccgtctcctc

SEQ ID NO: 146 - protein, 121 aa, Artificial
  Antibody
QVQLQESGPGLVKPSQTLSLTCTVSGGSISSGDYYWSWIRQYPGKGLEWIGYIYYSGSTYYNPSLKSRVTISVDTSKNQFSLKLGSVTAADTAVYFCARADYDFWSGYFDFWGQGTLVTVS

SEQ ID NO: 147 - DNA, 322 bp, Artificial
  Antibody
gacatccagatgacccagtctccatcctccctgtctgcatctgtaggagacagagtcaccatcacttgccgggcaagtcagggcattagaaatgatttaggctggtatcagcagaaaccagggaaagcccctaagcgcctgatctatgctgcatccagtttgcaaagtggggtcccatcaaggttcagcggcagtggatctgggacagaattcactctcacaatcagcagcctgcagcctgaagattttgcaacttattactgtctacagcataatggttacccgtggacgttcggccaagggaccaaggtggaaatcaaac

SEQ ID NO: 148 - protein, 107 aa, Artificial
  Antibody
DIQMTQSPSSLSASVGDRVTITCRASQGIRNDLGWYQQKPGKAPKRLIYAASSLQSGVPSRFSGSGSGTEFTLTISSLQPEDFATYYCLQHNGYPWTFGQGTKVEIK

SEQ ID NO: 149 - DNA, 365 bp, Artificial; identical to SEQ ID NO: 145
  Antibody

SEQ ID NO: 150 - protein, 121 aa, Artificial; identical to SEQ ID NO: 146
  Antibody

SEQ ID NO: 151 - DNA, 322 bp, Artificial; identical to SEQ ID NO: 147
  Antibody

SEQ ID NO: 152 - protein, 107 aa, Artificial; identical to SEQ ID NO: 148
  Antibody

SEQ ID NO: 153 - DNA, 366 bp, Artificial
  Antibody
caggtgcagctgcaggagtcgggcccaggactggtgaagccttcacagaccctgtccctcacctgcactgtctctggtggctccatcagtagtggtgattactactggagctggatccgccagcacccagggaagggcctggagtggattgggtacatctattacagtgggagcacctactacaacccgtccctcaagagtcgagttaccatatcagtagacacgtctaagaaccagttctccctgaagctgagctctgtgactgccgcggacacggccgtgtattactgtgcgagagcggattacgatttttggagtggttattttgactcctggggccagggaaccctggtcaccgtctcctca

SEQ ID NO: 154 - protein, 122 aa, Artificial
  Antibody
QVQLQESGPGLVKPSQTLSLTCTVSGGSISSGDYYWSWIRQHPGKGLEWIGYIYYSGSTYYNPSLKSRVTISVDTSKNQFSLKLSSVTAADTAVYYCARADYDFWSGYFDSWGQGTLVTVSS

SEQ ID NO: 155 - DNA, 321 bp, Artificial
  Antibody
gacatccagatgacccagtctccatcctccctgtctgcatctgtaggagacagagtcaccatcacttgccgggcaagtcagggcattagaaatgatttaggctggtatcagcagatacctgggaaagcccctaagcgcctgatctatgctgcatccagtttgcaaagtggggtcccatcaaggttcagcggcagtggatctgggacagaattcactctcacaatcagcagcctgcagcctgaagattttgcaacttattactgtctacagcataatggttacccgtggacgttcggccaagggaccaaggtggaaatcaaa

SEQ ID NO: 156 - protein, 107 aa, Artificial
  Antibody
DIQMTQSPSSLSASVGDRVTITCRASQGIRNDLGWYQQIPGKAPKRLIYAASSLQSGVPSRFSGSGSGTEFTLTISSLQPEDFATYYCLQHNGYPWTFGQGTKVEIK

SEQ ID NO: 157 - DNA, 366 bp, Artificial
  Antibody
caggttcagctggtgcagtctggagctgaggtgaagaagcctggggcctcagtgaaggtctcctgcaaggcttctggttacacctttaccaactatggtatcagctgggtgcggcaggcccctggacaagggcttgagtggatgggatggatcagcgcttacgatggttacagaaactatgcacagaagctccagggcagagtcaccatgaccacagacacatccacgaccactgcctacatggagctgaggagcctgagatctgacgacacggccgtgtattactgtgcgagagatgttcaagactacggtgactacgactactttgactactggggccagggaaccctggtcaccgtctcctca

SEQ ID NO: 158 - protein, 122 aa, Artificial
  Antibody
QVQLVQSGAEVKKPGASVKVSCKASGYTFTNYGISWVRQAPGQGLEWMGWISAYDGYRNYAQKLQGRVTMTTDTSTTTAYMELRSLRSDDTAVYYCARDVQDYGDYDYFDYWGQGTLVTVSS

SEQ ID NO: 159 - DNA, 321 bp, Artificial
  Antibody
gacatccagatgacccagtctccatcctccctgtctgcatctgtaggagacagagtcaccatcacttgccgggcaagtcagagcattagcagttatttaaattggtatcagcagaaaccagggaaagcccctaacctcctgatctatgctgcatccagtttgcaaagtggggtcccatcaagattcaggggcagtggatctgggacagatttcactctcaccatcagcagtctgcaacctgaagattttgcaacttactactgtcaacagagttacagtacccccatcaccttcggccaagggacacgactggagattaaa

SEQ ID NO: 160 - protein, 107 aa, Artificial
  Antibody
DIQMTQSPSSLSASVGDRVTITCRASQSISSYLNWYQQKPGKAPNLLIYAASSLQSGVPSRFRGSGSGTDFTLTISSLQPEDFATYYCQQSYSTPITFGQGTRLEIK

SEQ ID NO: 161 - DNA, 366 bp, Artificial
  Antibody
caggtgcagctgcaggagtcgggcccaggactggtgaagcctttacagaccctgtccctcacctgcactgtctctggtggctccatcagcagtggtgattactactggagctggatccgccagcacccagggaagggcctggagtggattgggtacatctattacagtgggaccacctactacaacccgtccctcaagagtcgagttaccatatcagtagacacgtctaagaaccagttcgccctgaagctgaactctgtgactgccgcggacacggccgtgtattactgtgcgagagccgattacgatttttggagtggttattttgactactggggccagggaaccctggtcaccgtctcctca

SEQ ID NO: 162 - protein, 122 aa, Artificial
  Antibody
QVQLQESGPGLVKPLQTLSLTCTVSGGSISSGDYYWSWIRQHPGKGLEWIGYIYYSGTTYYNPSLKSRVTISVDTSKNQFALKLNSVTAADTAVYYCARADYDFWSGYFDYWGQGTLVTVSS

SEQ ID NO: 163 - DNA, 322 bp, Artificial
  Antibody
gacatccagatgacccagtctccatcctccctgtctgcatctgtaggagacagagtcaccatcacttgccgggcaggtcagggcattagaaatgatttaggctggtatcagcagaaaccagggaaagcccctcagcgcctgatctatgctgcatccagtttgcaaagtggggtcccatcaaggttcagcggcagtggatctgggacagaattctctctcacaatctccagcctgcagcctgaagattttgcaacttattactgtctacagcataatagttacccgtggacgttcggccaagggaccaaggtggaaatcaaac

SEQ ID NO: 164 - protein, 107 aa, Artificial
  Antibody
DIQMTQSPSSLSASVGDRVTITCRAGQGIRNDLGWYQQKPGKAPQRLIYAASSLQSGVPSRFSGSGSGTEFSLTISSLQPEDFATYYCLQHNSYPWTFGQGTKVEIK

SEQ ID NO: 165 - DNA, 369 bp, Artificial
  Antibody
caggtgcagctggtggagtctgggggaggcttggtcaagcctggagggtccctgagactctcctgtgcagcctctggattcaccttcagtgactactacatgagctggatccgccaggctccagggaaggggctggagtgggtttcatatattagtagtagtggtaataacatataccacgcagactctgtgaagggccgattcaccatctccagggacaacgccaagaactcactgtatctgcaaatgaacagcctgagagccgaggacacggccgtgtattactgtgcgagagagagatatagtggctacgacgaccctgatggttttgatatctggggccaagggacaatggtcaccgtctcttca

SEQ ID NO: 166 - protein, 123 aa, Artificial
  Antibody
QVQLVESGGGLVKPGGSLRLSCAASGFTFSDYYMSWIRQAPGKGLEWVSYISSSGNNIYHADSVKGRFTISRDNAKNSLYLQMNSLRAEDTAVYYCARERYSGYDDPDGFDIWGQGTMVTVSS

SEQ ID NO: 167 - DNA, 321 bp, Artificial
  Antibody
gacatccagatgacccagtctccatcctccctgtctgcatctgtaggagacagagtcaccatcacttgccaggcgagtcaggacattagcaactatttaagttggtttcagcagaaaccagggaaagcccctaagctcctgatccacgatgcatccaatttggaaacaggggtcccttcaaggttcagtggaagtggatctgggacagattttactttcaccatcagcagcctgcagcctgaagatattgcaacatattactgtcaacagtatgataatcccccgtgcagttttggccaggggaccaagctggagatcaaa

SEQ ID NO: 168 - protein, 107 aa, Artificial
  Antibody
DIQMTQSPSSLSASVGDRVTITCQASQDISNYLSWFQQKPGKAPKLLIHDASNLETGVPSRFSGSGSGTDFTFTISSLQPEDIATYYCQQYDNPPCSFGQGTKLEIK

SEQ ID NO: 169 - DNA, 366 bp, Artificial
  Antibody
caggtgcagctgcaggagtcgggcccaggactggtgaagccttcacagaccctgtccctcacctgcactgtctctggtggctccatcagcagtggttattactactggagctggatccgccagcacccagggaagggcctggagtggattgggtacatctattacagtgggaccacctactacaatccgtccttcaagagtcgagttaccatatcagtagacacgtctaagaaccagttctccctgaaactgagctctgtgactgccgcggacacggccgtgtattactgtgcgagagccgattacgatttttggagtggtcactttgactactggggccagggaaccctggtcaccgtctcctca

SEQ ID NO: 170 - protein, 122 aa, Artificial
  Antibody
QVQLQESGPGLVKPSQTLSLTCTVSGGSISSGYYYWSWIRQHPGKGLEWIGYIYYSGTTYYNPSFKSRVTISVDTSKNQFSLKLSSVTAADTAVYYCARADYDFWSGHFDYWGQGTLVTVSS

SEQ ID NO: 171 - DNA, 321 bp, Artificial
  Antibody
gacatccagatgacccagtctccatcctccctgtctgcatctgtaggagacagagtcaccatcacttgccgggcaagtcagggcattagaaatgatttaggctggtatcagcagaaaccagggaaagcccctaagcgcctgatctatgctgcatccagtttgcaaagtggggtcccatcaaggttcagcggcagtggatctgggacagaattcactctcacaatcagcagcctgcagcctgaagattttgcaacttattactgtctacagcataatagttacccgtggacgttcggccaagggaccaaggtggaaatcaaa

SEQ ID NO: 172 - protein, 107 aa, Artificial; identical to SEQ ID NO: 136
  Antibody

SEQ ID NO: 173 - DNA, 365 bp, Artificial
  Antibody
caggttcagctggtgcagtctggagctgaggtgaagaagcctggggcctcagtgaaggtctcctgcaaggcttctggttacacctttaccagctatggtatcagctgggtgcgacaggcccctggacaaggacttgagtggatgggatggatcagcgcttacgatggtcacacaaactatgcacagaagctccagggcagagtcaccatgaccacagacacatccacgaacacagcctacatggagctgaggagcctgagatctgacgacacggccgtttattactgtgcgagagacccccatgactacagtaactacgaggcttttgacttctggggccagggaaccctggtcaccgtctcctc

SEQ ID NO: 174 - protein, 121 aa, Artificial
  Antibody
QVQLVQSGAEVKKPGASVKVSCKASGYTFTSYGISWVRQAPGQGLEWMGWISAYDGHTNYAQKLQGRVTMTTDTSTNTAYMELRSLRSDDTAVYYCARDPHDYSNYEAFDFWGQGTLVTVS

SEQ ID NO: 175 - DNA, 519 bp, Artificial
  Antibody
atgaggtcccctgctcagctcctggggctcctgctactctggctccgaggtgccagatgtgacatccagatgacccagtctccatcctccctgtctgcatctgtaggagacagagtcaccatcacttgccgggcaagtcagagcattagcagttatttaaattggtatcagcagaaaccagggaaagcccctaacctcctgatctatgctgcatccagtttgcaaagtggggtcccatcaagattcagtggcagtggatctgggacagatttcactctcaccatcagcagtctgcaacctgaagattttgcaacttactactgtcaacagagttacagtacccccatcaccttcggccaagggacacgactggagattaaacgaactgtggctgcaccatctgtcttcatcttcccgccatctgatgagcagttgaaatctggaactgcctctgttgtgtgcctgctgaataacttctatcccagagaggccaaagtacagtggaaggtggataacgcc

SEQ ID NO: 176 - protein, 107 aa, Artificial
  Antibody
DIQMTQSPSSLSASVGDRVTITCRASQSISSYLNWYQQKPGKAPNLLIYAASSLQSGVPSRFSGSGSGTDFTLTISSLQPEDFATYYCQQSYSTPITFGQGTRLEIK

SEQ ID NO: 177 - DNA, 534 bp, Artificial
  Antibody
accatggactggacctggagggtccttttcttggtggcagcagcaacaggtgcccactcccaggttcagctggtgcagtctggagctgaggtgaagaagcctggggcctcagtgaaggtctcctgcaaggcttctggttacacctttaccaactatggtatcagctgggtgcggcaggcccctggacaagggcttgagtggatgggatggatcagcgcttacgatggttacagaaactatgcacagaagctccagggcagagtcaccatgaccacagacacatccacgaccactgcctacatggagctgaggagcctgagatctgacgacacggccgtgtattactgtgcgagagatgttcaagactacggtgactacgactactttgactactggggccagggaaccctggtcaccgtctcctcagcttccaccaagggcccatccgtcttccccctggtgccctgctccaggagcacctccgagagcacagccgccctgggctgcctggtcaaggactacttccccgaaccg

SEQ ID NO: 178 - protein, 122 aa, Artificial; identical to SEQ ID NO: 158
  Antibody

SEQ ID NO: 179 - DNA, 504 bp, Artificial
  Antibody
cagctcctggggctcctgctactctggctccgaggtgccagatgtgacatccagatgacccagtctccatcctccctgtctgcatctgtaggagacagagtcaccatcacttgccgggcaagtcagagcattagcagttatttaaattggtatcagcagaaaccagggaaagcccctaacctcctgatctatgctgcatccagtttgcaaagtggggtcccatcaagattcagtggcagtggatctgggacagatttcactctcaccatcagcagtctgcaacctgaagattttgcaacttactactgtcaacagagttacagtacccccatcaccttcggccaagggacacgactggagattaaacgaactgtggctgcaccatctgtcttcatcttcccgccatctgatgagcagttgaaatctggaactgcctctgttgtgtgcctgctgaataacttctatcccagagaggccaaagtacagtggaaggtggataacgcc

SEQ ID NO: 180 - protein, 107 aa, Artificial; identical to SEQ ID NO: 176
  Antibody

SEQ ID NO: 181 - DNA, 493 bp, Artificial
  Antibody
catctgtggttcttcctcctgctggtggcagctcccagatgggtcctgtcccaggtgcagctgcaggagtcgggcccaggactggtgaagccttcacagaccctgtccctcacctgcactgtctctggtggctccatcaacagtggtgattactactggagctggatccgccagcacccagggaagggcctggagtggattgggtacatctattacagtgggagcacctactacaacccgtccctcaagagtcgagttaccatatcagtagacacgtctaagaaccagttctccctgaagctgagctctgtgactgccgcggacacggccgtgtattactgtgcgagagcagattacgatttttggagtggttactttgactactggggccagggaaccctggtcaccgtctcctcagcctccaccaagggcccatcggtcttccccctggcaccctcctccaagagcacctctgggggcacaacggccctgg

SEQ ID NO: 182 - protein, 122 aa, Artificial
  Antibody
QVQLQESGPGLVKPSQTLSLTCTVSGGSINSGDYYWSWIRQHPGKGLEWIGYIYYSGSTYYNPSLKSRVTISVDTSKNQFSLKLSSVTAADTAVYYCARADYDFWSGYFDYWGQGTLVTVSS

SEQ ID NO: 183 - DNA, 518 bp, Artificial
  Antibody
atgagggtccctgctcagctcctggggctcctgctgctctggttcccaggtgccaggtgtgacatccagatgacccagtctccatcctccctgtctgcatctgtaggagacagagtcaccatcacttgccgggcaagtcagggcattagaaatgatttaggctggtatcagcagaaaccagggaaagcccctaagcgcctgatctatgctgcatccagtttgcaaagtggggtcccatcaaggttcagcggcagtggatctgggacagaattcactctcacaatcagcagcctgcagcctgaagattttgcaacttattactgtctacagcataatagttacccgtggacgttcggccaagggaccaaggtggaaatcaaacgaactgtggctgcaccatctgtcttcatcttcccgccatctgatgagcagttgaaatctggaactgcctctgttgtgtgcctgctgaataacttctatcccagagaggccaaagtacagtggaaggtggataacgc

SEQ ID NO: 184 - protein, 107 aa, Artificial; identical to SEQ ID NO: 136
  Antibody

SEQ ID NO: 185 - DNA, 436 bp, Artificial
  Antibody
tggttcttccttctgctggtggcagctcccagatgggtcctgtcccaggtgcagctgcaggagtcgggcccaggactggtgaagccttcacagaccctgtccctcacctgcactgtctctggtggctccatcagcagtggtggttactactggagctggatccgccagcacccagggaagggcctggagtggattgggtacatctattacagtgggagcacctactacaacccgtccctcaagagtcgagttaccatatcagtagacacgtctaagaaccagttctccctgaagctgagctctgtgactgccgcggacacggccgtgtattactgtgcgagagatggctatgatagtagtggttattaccacggctactttgactactggggccagggaaccctggtcaccgtctcctcagcctccaccaagggcc

SEQ ID NO: 186 - protein, 125 aa, Artificial
  Antibody
QVQLQESGPGLVKPSQTLSLTCTVSGGSISSGGYYWSWIRQHPGKGLEWIGYIYYSGSTYYNPSLKSRVTISVDTSKNQFSLKLSSVTAADTAVYYCARDGYDSSGYYHGYFDYWGQGTLVTVSS

SEQ ID NO: 187 - DNA, 521 bp, Artificial
  Antibody
caggtcttcatttctctgttgctctggatctctggtgcctacggggacatcgtgatgacccagtctccagactccctggctgtgtctctgggcgagagggccaccatcaactgcaagtccagccagagtgttttatacagctccaacaataagaactacttagcttggtaccagcagaaaccaggacagcctcctaagctgctcatttactgggcatctacccgggaatccggggtccctgaccgattcagtggcagcgggtctgggacagatttcactctcaccatcagcagcctgcaggctgaagatgtggcagtttattactgtcagcaatattatagtactccgctcactttcggcggagggaccaaggtggagatcaaacgaactgtggctgcaccatctgtcttcatcttcccgccatctgatgagcagttgaaatctggaactgcctctgttgtgtgcctgctgaataacttctatcccagagaggccaaagtacagtggaaggtggataacgc

SEQ ID NO: 188 - protein, 113 aa, Artificial
  Antibody
DIVMTQSPDSLAVSLGERATINCKSSQSVLYSSNNKNYLAWYQQKPGQPPKLLIYWASTRESGVPDRFSGSGSGTDFTLTISSLQAEDVAVYYCQQYYSTPLTFGGGTKVEIK

SEQ ID NO: 189 - DNA, 455 bp, Artificial
  Antibody
ctgtggttcttcctcctgctggtggcagctcccagatgggtcctgtcccaggtgcagctgcaggagtcgggcccaggactggtgaagccttcacagaccctgtccctcacctgcactgtctctggtggctccatcagtagtggtgattactactggagctggatccgccagcacccagggaagggcctggagtggattgggtacatctattacagtgggagcacctactacaacccgtccctcaagagtcgagttaccatatcagtagacacgtctaagaaccagttctccctgaagttgagctctgtgactgccgcggacacggccgtgtattactgtgcgagagccgattacgatttttggagtggttattttgactactggggccagggaaccctggtcaccgtctcctcagcctccaccaagggcccatcggtcttccccctggcaccctc

SEQ ID NO: 190 - protein, 122 aa, Artificial; identical to SEQ ID NO: 92
  Antibody

SEQ ID NO: 191 - DNA, 442 bp, Artificial
  Antibody
gtgcccgctcagcgcctggggctcctgctgctctggttcccaggtgccaggtgtgacatccagatgacccagtctccatcctccctgtctgcatctgtaggagacagagtcaccatcacttgccgggcaagtcagggcattagaaatgatttaggctggtatcagcagaaaccagggaaagcccctaagcgcctgatctatgctgcatccagtttgcaaagtggggtcccatcaaggttcagcggcagtggatctgggacagaattcactctcacaatcagcagcctgcagcctgaagattttgcaacttattactgtctacagcataataattacccgtggacgttcggccaagggaccaaggtggaaatcaaacgaactgtggctgcaccatctgtcttcatcttcccgccatctgatgagcagttgaaatctggaactg

SEQ ID NO: 192 - protein, 107 aa, Artificial; identical to SEQ ID NO: 102
  Antibody

SEQ ID NO: 193 - DNA, 427 bp, Artificial
  Antibody
tggttcttccttctgctggtggcagctcccagatgggtcctgtcccaggtgcagctgcaggagtcgggcccaggactggtgaagccttcacagaccctgtccctcacctgcactgtctctggtggctccatcagcagtggtgattactactggagctggatccgccagcacccagggaagggcctggagtggattgggtacatctattacagtgggagcacctactacaacccgtccctcaagagtcgagttaccatatcagtagacacgtctaagaaccagttctccctgaagctgagctctgtgactgccgcggacacggccgtgtatttctgtgcgagagccgattacgatttttggagtggttattttgactactggggccagggaaccctggtcaccgtctcctcagcctccaccaagggcc

SEQ ID NO: 194 - protein, 122 aa, Artificial
  Antibody
QVQLQESGPGLVKPSQTLSLTCTVSGGSISSGDYYWSWIRQHPGKGLEWIGYIYYSGSTYYNPSLKSRVTISVDTSKNQFSLKLSSVTAADTAVYFCARADYDFWSGYFDYWGQGTLVTVSS

SEQ ID NO: 195 - DNA, 518 bp, Artificial
  Antibody
atgagggtccccgctcagctcctggggctcctgctgctctggttcccaggtgccaggtgtgacatccagatgacccagtctccatcctccctgtctgcatctgtaggagacagagtcaccatcacttgccgggcaagtcagggcattagaaatgatttaggctggtatcagcagaaaccagggaaagcccctaagcgcctgatctatgctgcatccagtttgcaaagtggggtcccatcaaggttcagcggcagtggatctgggacagaattcactctcacaatcagcagcctgcagcctgaagattttgcaacttattactgtctacagcataatacttacccgtggacgttcggccaagggaccaaggtggaaatcaaacgaactgtggctgcaccatctgtcttcatcttcccgccatctgatgagcagttgaaatctggaactgcctctgttgtgtgcctgctgaataacttctatcccagagaggccaaagtacagtggaaggtggataacgc

SEQ ID NO: 196 - protein, 107 aa, Artificial; identical to SEQ ID NO: 114
  Antibody

SEQ ID NO: 197 - DNA, 428 bp, Artificial
  Antibody
tggttcttccttctgctggtggcagctcccagatgggtcctgtcccaggtgcagctgcaggagtcgggcccaggactggtgaagccttcacagaccctgtccctcacctgcactgtctctggtggctccatcagcagtggtgattactactggagctggatccgccagcacccagggaagggcctggagtggattgggtacatctattacagtgggagcacctactacaacccgtccctcaagagtcgagttaccatatcagtagacacgtctaagaaccagttctccctgaagctgagctctgtgactgccgcggacacggccgtgtatttctgtgcgagagccgattacgatttttggaatggttattttgactactggggccagggaaccctggtcaccgtctcctcagcctccaccaagggccc

SEQ ID NO: 198 - protein, 122 aa, Artificial
  Antibody
QVQLQESGPGLVKPSQTLSLTCTVSGGSISSGDYYWSWIRQHPGKGLEWIGYIYYSGSTYYNPSLKSRVTISVDTSKNQFSLKLSSVTAADTAVYFCARADYDFWNGYFDYWGQGTLVTVSS

SEQ ID NO: 199 - DNA, 519 bp, Artificial
  Antibody
atgagggtccccgctcagctcctggggctcctgctgctctggttcccaggtgccaggtgtgacatccagatgacccagtctccatcctccctgtctgcatctgtaggagacagagtcaccatcacttgccgggcaagtcagggcattagaaatgatttaggctggtatcagcagaaaccagggaaagcccctaagcgcctgatctatgctgcttccagtttgcaaagtggggtcccatcaaggttcagcggcagtggatctgggacagaattcactctcacaatcagcagcctgcagcctgaagattttgcaacttattactgtctacagcataatacttacccgtggacgttcggccaagggaccaaggtggaaatcaaacgaactgtggctgcaccatctgtcttcatcttcccgccatctgatgagcagttgaaatctggaactgcctctgttgtgtgcctgctgaataacttctatcccagagaggccaaagtacagtggaaggtggataacgcc

SEQ ID NO: 200 - protein, 107 aa, Artificial; identical to SEQ ID NO: 114
  Antibody

SEQ ID NO: 201 - DNA, 398 bp, Artificial
  Antibody
ttggtggcagcagctacaggcacccacgcccaggtccagctggtacagtctggggctgaggtgaagaagcctggggcctcagtgaaggtctcctgcaaggtttccggatacaccctcactgaattatccatgtactgggtgcgacaggctcctggaaaagggcttgagtggatgggaggttttgatcctgaagatggtgaaacaatctacgcacagaagttccagggcagagtcaccatgaccgaggacacatctacagacacagcctacatggagctgagcagcctgagatctgaggacacggccgtgtattactgtgcaactgggtggaactacgtctttgactactggggccagggaaccctggtcaccgtctcctcagcctccaccaagggccc

SEQ ID NO: 202 - protein, 117 aa, Artificial
  Antibody
QVQLVQSGAEVKKPGASVKVSCKVSGYTLTELSMYWVRQAPGKGLEWMGGFDPEDGETIYAQKFQGRVTMTEDTSTDTAYMELSSLRSEDTAVYYCATGWNYVFDYWGQGTLVTVSS

SEQ ID NO: 203 - DNA, 388 bp, Artificial
  Antibody
ggatccagtggggatattgtgatgactcagtctccactctccctgcccgtcacccctggagagccggcctccatctcctgcaggtccagtcagagcctcctgcatagtaatggatacaactatttggattggtacctgcagaagccagggcagtctccacagctcctgatctatttggattctcatcgggcctccggggtccctgacaggttcagtggcagtggatcaggcacagattttacactgaaaatcagcagagtggaggctgaggatgttggggtttattactgcatgcaagctctacaaactccgctcactttcggcggagggaccaaggtggagatcaaacgaactgtggctgcaccatctgtcttcatcttcccgccat

SEQ ID NO: 204 - protein, 112 aa, Artificial
  Antibody
DIVMTQSPLSLPVTPGEPASISCRSSQSLLHSNGYNYLDWYLQKPGQSPQLLIYLDSHRASGVPDRFSGSGSGTDFTLKISRVEAEDVGVYYCMQALQTPLTFGGGTKVEIK

SEQ ID NO: 205 - DNA, 446 bp, Artificial
  Antibody
tggttcttccttctgctggtggcagctcccagatgggtcctgtcccaggtgcagctgcaggagtcgggcccaggactggtgaagccttcacagaccctgtccctcacctgcactgtctctggtggctccatcagcagtggtgattactactggagctggatccgccagcacccagggaagggcctggagtggattgggtacatctattacagtgggagcacctactacaacccgtccctcaagagtcgagttaccatatcagtagacacgtctaagaaccagttctccctgaagctgagctctgtgactgccgcggacacggccgtgtatttctgtgcgagagccgattacgatttttggagtggttattttgactactggggccagggaaccctggtcaccgtctcctcagcctccaccaagggcccatcgagtcttccccctgg

SEQ ID NO: 206 - protein, 122 aa, Artificial; identical to SEQ ID NO: 194
  Antibody

SEQ ID NO: 207 - DNA, 519 bp, Artificial
  Antibody
atgagggtccccgctcagctcctggggctcctgctgctctggttcccaggtgccaggtgtgacatccagatgacccagtctccatcctccctgtctgcatctgtaggagacagagtcaccatcacttgccgggcaagtcagggcattagaaatgatttaggctggtatcagcagaaaccagggaaagcccctaagcgcctgatctatgctgcatccagtttgcaaagtggggtcccatcaaggttcagcggcagtggatctgggacaaaattcactctcactatcagcagcctgcagcctgaagattttgcaacttattactgtctacagcataatacttacccgtggacgttcggccaagggaccaaggtggaaatcagacgaactgtggctgcaccatctgtcttcatcttcccgccatctgatgagcagttgaaatctggaactgcctctgttgtgtgcctgctgaataacttctatcccagagaggccaaagtacagtggaaggtggataacgcc

SEQ ID NO: 208 - protein, 107 aa, Artificial
  Antibody
DIQMTQSPSSLSASVGDRVTITCRASQGIRNDLGWYQQKPGKAPKRLIYAASSLQSGVPSRFSGSGSGTKFTLTISSLQPEDFATYYCLQHNTYPWTFGQGTKVEIR

SEQ ID NO: 209 - DNA, 564 bp, Artificial
  Antibody
accatgaaacatctgtggttcttcctcctgctggtggcagctcccagatgggtcctgtcccaggtgcagctgcaggagtcgggcccaggactggtgaagccttcacagaccctgtccctcacctgcactgtctctggtggctccatcagcagtggtgattactactggagctggatccgccagcacccagggaagggcctggagtggattgggtacatctattacagtgggagcacctactacaacccgtccctcaagagtcgagttaccatatcagtagacacgtctaagaaccagttctccctgaagctgagctctgtgactgccgcggacacggccgtgtattactgtgcgagagcggattacgatttttggagtggttattttgactactggggccagggaatcctggtcaccgtctcctcagcctccaccaagggcccatcggtcttccccctggcaccctcctccaagaacacctctgggggcacagcggccctgggctgcctggtcaaggactacttccccgaaccggtgacggtgtcctggaactcaggcgccctg

SEQ ID NO: 210 - protein, 122 aa, Artificial
  Antibody
QVQLQESGPGLVKPSQTLSLTCTVSGGSISSGDYYWSWIRQHPGKGLEWIGYIYYSGSTYYNPSLKSRVTISVDTSKNQFSLKLSSVTAADTAVYYCARADYDFWSGYFDYWGQGILVTVSS

SEQ ID NO: 211 - DNA, 519 bp, Artificial
  Antibody
atgagggtccccgctcagctcctggggctcctgctgctctggttcccaggtgccaggtgtgacatccagatgacccagtctccatcctccctgtctgcatctgtaggagacagagtcaccatcacttgccgggcaagtcagggcattagaaatgatttaggctggtatcagcagaaaccagggaaagcccctaagcgcctgatctatgctgcatccagtttgcaaagtggggtcccatcaaggttcagcggcagtggatctgggacagaattcactctcacaatcagcagcctgcagcctgaagattttgcaacttattactgtctacagcataatagttacccgtggacgttcggccaagggaccaaggtggaaatcaaacgaactgtggctgcaccatctgtcttcatcttcccgccatctgatgagcagttgaaatctggaactgcctctgttgtgtgcctgctgaataacttctatcccagagaggccaaagtacagtggaaggtggataacgcc

SEQ ID NO: 212 - protein, 107 aa, Artificial; identical to SEQ ID NO: 136
  Antibody

SEQ ID NO: 213 - DNA, 432 bp, Artificial
  Antibody
tggttcttccttctgctggtggcagctcccagatgggtcctgtcccaggtgcagctgcaggagtcgggcccaggactggtgaagccttcacagaccctgtccctcacctgcactgtctctggtggctccatcagcagtggtgattactactggagctggatccgccagcacccagggaagggcctggagtggattggatacatctattacagtgggagcacctactacaattcgtccctcaagagtcgagttaccatatcagtagacacgtctaagaaccagttctccctgaagctgagctctgtgactgccgcggacacggccgtgtattactgtgcgagagcggattacgatttttggagtggttattttgactactggggccagggaaccctggtcaccgtctcctcagcctccaccaagggcccatcg

SEQ ID NO: 214 - protein, 122 aa, Artificial
  Antibody
QVQLQESGPGLVKPSQTLSLTCTVSGGSISSGDYYWSWIRQHPGKGLEWIGYIYYSGSTYYNSSLKSRVTISVDTSKNQFSLKLSSVTAADTAVYYCARADYDFWSGYFDYWGQGTLVTVSS

SEQ ID NO: 215 - DNA, 372 bp, Artificial
  Antibody
ggtgccaggtgtgacatccagatgacccagtctccatcctccctgtctgcatctgtaggagacagagtcaccatcacttgccgggcaagtcagggcattagaaatgatttaggctggtatcagcagaaacctgggaaagcccctaagcgcctgatctatgctgcatccagtttgcaaagtggggtcccatcaaggttcagcggcagtggatctgggacagaattcactctcacaatcagcagcctgcagcctgaagattttgcaacttattactgtctacagcacaatagttacccgtggacgttcggccaagggaccaaggtggaaatcaaacgaactgtggctgcaccatctgtcttcatcttcccgcca

SEQ ID NO: 216 - protein, 107 aa, Artificial; identical to SEQ ID NO: 136
  Antibody

SEQ ID NO: 217 - DNA, 548 bp, Artificial
  Antibody
aggttcttccttctgctggtggcagctcccagatgggtcctgtcccaggtgcagctgcaggagtcgggcccaggactggtgaagccttcacagaccctgtccctcacctgcactgtctctggtggctccatcagcagtggtgattactactggagctggatccgccagcacccagggaagggcctggagtggattggatacatctattacagtgggagcacctactacaacccgtccctcaagagtcgagttaccatatcagtagacacgtctaagaaccagttctccctgaagctgagctctgtgactgccgcggacacggccgtgtattactgtgcgagagccgattacgatttttggagtggttattttgactactggggccagggaaccctggtcaccgtctcctcagcctccaccaagggcccatcggtcttccccctggcaccctcctccaagagcacctctgggggcacagcggccctgggctgcctggtcaaggactacttccccgaaccggtgacggtgtcgtggaactcaggcgccct

SEQ ID NO: 218 - protein, 122 aa, Artificial; identical to SEQ ID NO: 92
  Antibody

SEQ ID NO: 219 - DNA, 517 bp, Artificial
  Antibody
atgagggtccccgctcagctcctggggctcctgctgctctggttcccaggtgccaggtgtgacatccagatgacccagtctccatcctccctgtctgcatctgtaggagacagagtcaccatcacttgccgggcaagtcagggcattagaaatgatttaggctggtatcagcagaaaccagggaaagcccctaagcgcctgatctatgctgcatccagtttgcaaagtggggtcccatcaaggttcagcggcagtggatctgggacagaattcactctcacaatcagcagcctgcagcctgaagattttgcaacttattactgtctacagcataatagttacccgtggacgttcggccaagggaccaaggtggaaatcaaacgaactgtggctgcaccatctgtcttcatcttcccgccatctgatgagcagttgaaatctggaactgcctctgttgtgtgcctgctgaataacttctatcccagagaggccaaagtacagtggaaggtggataacg

SEQ ID NO: 220 - protein, 107 aa, Artificial; identical to SEQ ID NO: 136
  Antibody

SEQ ID NO: 221 - DNA, 446 bp, Artificial
  Antibody
ctgtggttcttccttctgctggtggcagctcccagatgggtcctgtcccaggtgcagctgcaggagtcgggcccaggactggtgaagccttcacagaccctgtccctcacctgcactgtctctggtggctccatcagcagtggtgattactactggagctggatccgccagcacccagggaagggcctggagtggattgggtacatctattacagtgggagcacctactacaacccgtccctcaagagtcgagttaccatgtcagtagacacgtctaagaaccagttctccctgaagctgagctctgtgactgccgcggacacggccgtgtattactgtgcgagagccgattacgatttttggagtggtcactttgactgctggggccagggaaccctggtcaccgtctcctcagcttccaccaagggccccatccgtcttccccc

SEQ ID NO: 222 - protein, 122 aa, Artificial
  Antibody
QVQLQESGPGLVKPSQTLSLTCTVSGGSISSGDYYWSWIRQHPGKGLEWIGYIYYSGSTYYNPSLKSRVTMSVDTSKNQFSLKLSSVTAADTAVYYCARADYDFWSGHFDCWGQGTLVTVSS

SEQ ID NO: 223 - DNA, 419 bp, Artificial
  Antibody
atgagggtccccgctcagctcctggggctcctgctgctctggttcccaggtgccaggtgtgacatccagatgacccagtctccatcctccctgtctgcatctgtaggagacagagtcaccatcacttgccgggcaagtcagggcattagagatgatttaggctggtatcagcagaaaccagggaaagcccctaagcgcctgatctatgctgaatccagtttgcaaagtggggtcccatcaaggttcagcggcagtggatctgggacagaattcactctcacaatcagcagcctgcagcctgaagattttgcaacttattactgtctacagcatcatagttacccgtggacgttcggccaagggaccaaggtggaaatcaaacgaactgtggctgcaccatctgtcttcatcttcccgcc

SEQ ID NO: 224 - protein, 107 aa, Artificial
  Antibody
DIQMTQSPSSLSASVGDRVTITCRASQGIRDDLGWYQQKPGKAPKRLIYAESSLQSGVPSRFSGSGSGTEFTLTISSLQPEDFATYYCLQHHSYPWTFGQGTKVEIK

SEQ ID NO: 225 - DNA, 504 bp, Artificial
  Antibody
tggctgagctgggttttcctcgttgctcttttaagaggtgtccagtgtcaggtgcagctggtggagtctgggggaggcgtggtccagcctgggaggtccctgagactctcctgtgcagcgtctggattcaccttcaatagctatgacatgcactgggtccgccaggctccaggcaaggggctggagtgggtggcagttatatggtatgatggaagtaataaatactatgcagactccgtgaagggccgattcaccatctctagagacaattccaagaacacgctgtatctgcaaatgaacagcctgagagccgaggacacggctgtgtattactgtgcgagagaccgcttgtgtactaatggtgtatgctatgaagactacggtatggacgtctggggccaagggaccacggtcaccgtctcctcagcttccaccaagggcccatccgtcttccccctggcgccctgctccaggagcacctccgagagcacagccgccctgggc

SEQ ID NO: 226 - protein, 126 aa, Artificial
  Antibody
QVQLVESGGGVVQPGRSLRLSCAASGFTFNSYDMHWVRQAPGKGLEWVAVIWYDGSNKYYADSVKGRFTISRDNSKNTLYLQMNSLRAEDTAVYYCARDRLCTNGVCYEDYGMDVWGQGTTVTVSS

SEQ ID NO: 227 - DNA, 504 bp, Artificial
  Antibody
atgagggtccctgctcagctcctggggctcctgctgctctggctctcaggtgccagatgtgacatccagatgacccagtctccatcctccctgtctgcatctgtaggagacagagtcaccatcacttgccaggcgagtcaggacattagcaactatttaaattggtatcagcagaaaccagggaaagcccctaaggtcctgatctacgatgcatccaatttggaaacaggggtcccatcaaggttcagtggaagtggatctgggacagattttactttcaccatcagcagcctgcagcctgaagatgttgcaacatattactgtcaacactatgatactctcccgctcactttcggcggagggaccaaggtggagatcaaacgaactgtggctgcaccatctgtcttcatcttcccgccatctgatgagcagttgaaatctggaactgcctctgttgtgtgcctgctgaataacttctatcccagagaggccaaagtacagtgg

SEQ ID NO: 228 - protein, 107 aa, Artificial
  Antibody
DIQMTQSPSSLSASVGDRVTITCQASQDISNYLNWYQQKPGKAPKVLIYDASNLETGVPSRFSGSGSGTDFTFTISSLQPEDVATYYCQHYDTLPLTFGGGTKVEIK

SEQ ID NO: 229 - DNA, 472 bp, Artificial
  Antibody
ggactgtgcaagaacatgaaacacctgtggttcttcctcctgctggtggcagctcccagatgggtcctgtcccaggtgcagctgcaggagtcgggcccaggactggtgaagcctttacagaccctgtccctcacctgcactgtctctggtggctccatcagcagtggtgattactactggagctggatccgccagcacccagggaagggcctggagtggattgggtacatctattacagtgggaccacctactacaacccgtccctcaagagtcgagttaccatatcagtagacacgtctaagaaccagttcgccctgaagctgaactctgtgactgccgcggacacggccgtgtattactgtgcgagagccgattacgatttttggagtggttattttgactactggggccagggaaccctggtcaccgtctcctcagcttccaccaagggcccatccgtcttccccctgg

SEQ ID NO: 230 - protein, 122 aa, Artificial; identical to SEQ ID NO: 162
  Antibody

SEQ ID NO: 231 - DNA, 531 bp, Artificial
  Antibody
atgagggtccctgctcagctcctggggctcctgctgctctggttcccaggtgccaggtgtgacatccagatgacccagtctccatcctccctgtctgcatctgtaggagacagagtcaccatcacttgccgggcaggtcagggcattagaaatgatttaggctggtatcagcagaaaccagggaaagcccctcagcgcctgatctatgctgcatccagtttgcaaagtggggtcccatcaaggttcagcggcagtggatctgggacagaattctctctcacaatctccagcctgcagcctgaagattttgcaacttattactgtctacagcataatagttacccgtggacgttcggccaagggaccaaggtggaaatcaaacgaactgtggctgcaccatctgtcttcatcttcccgccatctgatgagcagttgaaatctggaactgcctctgttgtgtgcctgctgaataacttctatcccagagaggccaaagtacagtggaaggtggataacgcccttccaatcggg

SEQ ID NO: 232 - protein, 107 aa, Artificial; identical to SEQ ID NO: 164
  Antibody

SEQ ID NO: 233 - DNA, 26 bp, Artificial
  Primer
  prim_transcript (1)..(26)
cgggatccatgtcctagcctaggggc

SEQ ID NO: 234 - DNA, 39 bp, Artificial
  Primer
  prim_transcript (1)..(39)
gctctagattaatgatgatgatgatgatgttgtcctaaa

SEQ ID NO: 235 - protein, 12 aa, Artificial
  U1-1 CDR-1-h
GGSINSGDYYWS

SEQ ID NO: 236 - protein, 16 aa, Artificial
  U1-1 CDR-2-h
YIYYSGSTYYNPSLKS

SEQ ID NO: 237 - protein, 12 aa, Artificial
  U1-1 CDR-3-h
ADYDFWSGYFDY

SEQ ID NO: 238 - protein, 11 aa, Artificial
  U1-1 CDR-1-l
RASQGIRNDLG

SEQ ID NO: 239 - protein, 7 aa, Artificial
  U1-1 CDR-2-l
AASSLQS

SEQ ID NO: 240 - protein, 9 aa, Artificial
  U1-1 CDR-3-l
LQHNSYPWT

SEQ ID NO: 241 - protein, 12 aa, Artificial
  U 1 - 2-CDR-1h
GGSISSGDYYWS

SEQ ID NO: 242 - protein, 16 aa, Artificial
  U 1 - 2-CDR-2h
YIYYSGSTYYNPSLRS

SEQ ID NO: 243 - protein, 12 aa, Artificial
  U 1 - 2-CDR-3h
ADYDFWSGYFDY

SEQ ID NO: 244 - protein, 11 aa, Artificial
  U 1 - 2-CDR-1l
RASQGIRNDLG

SEQ ID NO: 245 - protein, 7 aa, Artificial
  U 1 - 2-CDR-2l
AASSLQS

SEQ ID NO: 246 - protein, 9 aa, Artificial
  U 1 - 2-CDR-3l
LQHNGYPWT

SEQ ID NO: 247 - protein, 12 aa, Artificial
  U 1 - 3-CDR-1-h
GGSISSGGYYWS

SEQ ID NO: 248 - protein, 16 aa, Artificial
  U 1 - 3-CDR-2h
YIYYSGSTYYNPSLKS

SEQ ID NO: 249 - protein, 15 aa, Artificial
  U 1 - 3-CDR-3h
DGYDSSGYYHGYFDY

SEQ ID NO: 250 - protein, 17 aa, Artificial
  U 1 - 3-CDR-1l
KSSQSVLYSSNNKNYLA

SEQ ID NO: 251 - protein, 7 aa, Artificial
  U 1 - 3-CDR-2l
WASTRES

SEQ ID NO: 252 - protein, 9 aa, Artificial
  U 1 - 3-CDR-3l
QQYYSTPLT

SEQ ID NO: 253 - protein, 12 aa, Artificial
  U 1 - 4-CDR-1h
GGSISSGDYYWS

SEQ ID NO: 254 - protein, 16 aa, Artificial
  U 1 - 4-CDR-2h
YIYYSGSTYYNPSLKS

SEQ ID NO: 255 - protein, 12 aa, Artificial
  U 1 - 4-CDR-3h
ADYDFWSGYFDY

SEQ ID NO: 256 - protein, 11 aa, Artificial
  U 1 - 4-CDR-1l
RASQGIRNDLG

SEQ ID NO: 257 - protein, 7 aa, Artificial
  U 1 - 4-CDR-2l
AASSLQS

SEQ ID NO: 258 - protein, 9 aa, Artificial
  U 1 - 4-CDR-3l
LQHNNYPWT

SEQ ID NO: 259 - protein, 12 aa, Artificial
  U 1 - 5-CDR-1h
GGSISSGDYYWS

SEQ ID NO: 260 - protein, 16 aa, Artificial
  U 1 - 5-CDR-2h
YIYYSGSTYYNPSLKS

SEQ ID NO: 261 - protein, 12 aa, Artificial
  U 1 - 5-CDR-3h
ADYDFWSGYFDY

SEQ ID NO: 262 - protein, 11 aa, Artificial
  U 1 - 5-CDR-1l
RASQGIRNDLG

SEQ ID NO: 263 - protein, 7 aa, Artificial
  U 1 - 5-CDR-2l
AASSLQS

SEQ ID NO: 264 - protein, 9 aa, Artificial
  U 1 - 5-CDR-3l
LQHNTYPWT

SEQ ID NO: 265 - protein, 12 aa, Artificial
  U1-6-CDR-1h
GGSISSGDYYWS

SEQ ID NO: 266 - protein, 16 aa, Artificial
  U1-6-CDR-2h
YIYYSGSTYYNPSLKS

SEQ ID NO: 267 - protein, 12 aa, Artificial
  U1-6-CDR-3h
ADYDFWNGYFDY

SEQ ID NO: 268 - protein, 11 aa, Artificial
  U1-6-CDR-1l
RASQGIRNDLG

SEQ ID NO: 269 - protein, 7 aa, Artificial
  U1-6-CDR-2l
AASSLQS

SEQ ID NO: 270 - protein, 9 aa, Artificial
  U1-6-CDR-3l
LQHNTYPWT

SEQ ID NO: 271 - protein, 12 aa, Artificial
  U 1 - 7-CDR-1h
GGSISSGDYYWS

SEQ ID NO: 272 - protein, 16 aa, Artificial
  U 1 - 7-CDR-2h
YIYYSGSTYYNPSLKS

SEQ ID NO: 273 - protein, 12 aa, Artificial
  U 1 - 7-CDR-3h
ADYDFWSGYFDY

SEQ ID NO: 274 - protein, 11 aa, Artificial
  U 1 - 7-CDR-1l
RASQDIRNDLG

SEQ ID NO: 275 - protein, 7 aa, Artificial
  U 1 - 7-CDR-2l
AASSLQS

SEQ ID NO: 276 - protein, 9 aa, Artificial
  U 1 - 7-CDR-3l
LQHNSYPWT

SEQ ID NO: 277 - protein, 10 aa, Artificial
  U 1 - 8-CDR-1h
GYTLTELSMY

SEQ ID NO: 278 - protein, 17 aa, Artificial
  U 1 - 8-CDR-2h
GFDPEDGETIYAQKFQG

SEQ ID NO: 279 - protein, 8 aa, Artificial
  U 1 - 8-CDR-3h
GWNYVFDY

SEQ ID NO: 280 - protein, 16 aa, Artificial
  U 1 - 8-CDR-1l
RSSQSLLHSNGYNYLD

SEQ ID NO: 281 - protein, 7 aa, Artificial
  U 1 - 8-CDR-2l
LDSHRAS

SEQ ID NO: 282 - protein, 9 aa, Artificial
  U 1 - 8-CDR-3l
MQALQTPLT

SEQ ID NO: 283 - protein, 12 aa, Artificial
  U 1 - 9-CDR-1h
GGSISSGDYYWS

SEQ ID NO: 284 - protein, 16 aa, Artificial
  U 1 - 9-CDR-2h
YIYYSGSTYYNPSLKS

SEQ ID NO: 285 - protein, 12 aa, Artificial
  U 1 - 9-CDR-3h
ADYDFWNGYFDY

SEQ ID NO: 286 - protein, 11 aa, Artificial
  U 1 - 9-CDR-1l
RASQDIRNDLG

SEQ ID NO: 287 - protein, 7 aa, Artificial
  U 1 - 9-CDR-2l
AASSLQS

SEQ ID NO: 288 - protein, 9 aa, Artificial
  U 1 - 9-CDR-3l
LQHNSYPWT

SEQ ID NO: 289 - protein, 12 aa, Artificial
  U1-10-CDR-1h
GGSISSGDYYWS

SEQ ID NO: 290 - protein, 16 aa, Artificial
  U1-10-CDR-2h
YIYYSGSTYYNPSLKS

SEQ ID NO: 291 - protein, 12 aa, Artificial
  U1-10-CDR-3h
ADYDFWSGYFDY

SEQ ID NO: 292 - protein, 11 aa, Artificial
  U1-10-CDR-1l
RASQGIRNDLG

SEQ ID NO: 293 - protein, 7 aa, Artificial
  U1-10-CDR-2l
AASSLQS

SEQ ID NO: 294 - protein, 9 aa, Artificial
  U1-10-CDR-3l
LQHNNYPWT

SEQ ID NO: 295 - protein, 12 aa, Artificial
  U 1 -11-CDR-1h
GGSISSGDYYWS

SEQ ID NO: 296 - protein, 16 aa, Artificial
  U 1 -11-CDR-2h
YIYYSGSTYYNPSLKS

SEQ ID NO: 297 - protein, 12 aa, Artificial
  U 1 -11-CDR-3h
ADYDFWSGYFDY

SEQ ID NO: 298 - protein, 11 aa, Artificial
  U 1 -11-CDR-1l
RASQGIRNDLG

SEQ ID NO: 299 - protein, 7 aa, Artificial
  U 1 -11-CDR-2l
AASSLQS

SEQ ID NO: 300 - protein, 9 aa, Artificial
  U 1 -11-CDR-3l
LQHNTYPWT

SEQ ID NO: 301 - protein, 12 aa, Artificial
  U 1 - 12-CDR-1h
GGSISSGDYYWS

SEQ ID NO: 302 - protein, 16 aa, Artificial
  U 1 - 12-CDR-2h
YIYYSGSTYYNPSLKS

SEQ ID NO: 303 - protein, 12 aa, Artificial
  U1-12-CDR-3h
ADYDFWSGYFDY

SEQ ID NO: 304 - protein, 11 aa, Artificial
  U1-12-CDR-1l
RASQGIRNDLG

SEQ ID NO: 305 - protein, 7 aa, Artificial
  U1-12-CDR-2l
AASSLQS

SEQ ID NO: 306 - protein, 9 aa, Artificial
  U1-12-CDR-3l
LQHNNYPWT

SEQ ID NO: 307 - protein, 12 aa, Artificial
  U 1 -13-CDR-1h
GGSISSGGYYWS

SEQ ID NO: 308 - protein, 16 aa, Artificial
  U 1 -13-CDR-2h
YIYYSGSTYYNPSLKS

SEQ ID NO: 309 - protein, 7 aa, Artificial
  U 1 -13-CDR-3h
EDDGMDV

SEQ ID NO: 310 - protein, 16 aa, Artificial
  U 1 -13-CDR-1l
RSSQSLLHSNGYNYLE

SEQ ID NO: 311 - protein, 7 aa, Artificial
  U 1 -13-CDR-2l
LGSNRAS

SEQ ID NO: 312 - protein, 9 aa, Artificial
  U 1 -13-CDR-3l
MQALQTPIT

SEQ ID NO: 313 - protein, 12 aa, Artificial
  U1-14-CDR-1h
GGSISSGDYYWS

SEQ ID NO: 314 - protein, 16 aa, Artificial
  U1-14-CDR-2h
YIYYSGSTYYNPSLKS

SEQ ID NO: 315 - protein, 12 aa, Artificial
  U1-14-CDR-3h
ADYDFWSGYFDY

SEQ ID NO: 316 - protein, 11 aa, Artificial
  U1-14-CDR-1l
RASQGIRNDLG

SEQ ID NO: 317 - protein, 7 aa, Artificial
  U1-14-CDR-2l
AASSLQS

SEQ ID NO: 318 - protein, 9 aa, Artificial
  U1-14-CDR-3l
LQHNTYPWT

SEQ ID NO: 319 - protein, 12 aa, Artificial
  U1-15-CDR-1h
GGSVSSGGYYWS

SEQ ID NO: 320 - protein, 16 aa, Artificial
  U1-15-CDR-2h
YIYYSGSTNYNPSLKS

SEQ ID NO: 321 - protein, 14 aa, Artificial
  U1-15-CDR-3h
DGDVDTAMVDAFDI

SEQ ID NO: 322 - protein, 12 aa, Artificial
  U1-15-CDR-1l
RASQSLSGNYLA

SEQ ID NO: 323 - protein, 7 aa, Artificial
  U1-15-CDR-2l
GASSRAT

SEQ ID NO: 324 - protein, 9 aa, Artificial
  U1-15-CDR-3l
QQYDRSPLT

SEQ ID NO: 325 - protein, 12 aa, Artificial
  U1-16-CDR-1h
GGSISSGDYYWS

SEQ ID NO: 326 - protein, 16 aa, Artificial
  U1-16-CDR-2h
YIYYSGSTYYNPSLKS

SEQ ID NO: 327 - protein, 12 aa, Artificial
  U1-16-CDR-3h
ADYDFWSGYFDY

SEQ ID NO: 328 - protein, 11 aa, Artificial
  U1-16-CDR-1l
RASQGIRNDLG

SEQ ID NO: 329 - protein, 7 aa, Artificial
  U1-16-CDR-2l
AASSLQS

SEQ ID NO: 330 - protein, 9 aa, Artificial
  U1-16-CDR-3l
LQHNSYPWT

SEQ ID NO: 331 - protein, 12 aa, Artificial
  U1-17-CDR-1h
GGSISSGDYYWS

SEQ ID NO: 332 - protein, 16 aa, Artificial
  U1-17-CDR-2h
YIYYSGSTYYNSSLKS

SEQ ID NO: 333 - protein, 12 aa, Artificial
  U1-17-CDR-3h
ADYDFWSGYFDY

SEQ ID NO: 334 - protein, 11 aa, Artificial
  U1-17-CDR-1l
RASQGIRNDLG

SEQ ID NO: 335 - protein, 7 aa, Artificial
  U1-17-CDR-2l
AASSLQS

SEQ ID NO: 336 - protein, 9 aa, Artificial
  U1-17-CDR-3l
LQHNSYPWT

SEQ ID NO: 337 - protein, 12 aa, Artificial
  U1-18-CDR-1h
GGSISSGDYYWS

SEQ ID NO: 338 - protein, 16 aa, Artificial
  U1-18-CDR-2h
YIYYSGSTYYNPSLKS

SEQ ID NO: 339 - protein, 12 aa, Artificial
  U1-18-CDR-3h
ADYDFWSGYFDY

SEQ ID NO: 340 - protein, 11 aa, Artificial
  U1-18-CDR-1l
RASQGIRNDLG

SEQ ID NO: 341 - protein, 7 aa, Artificial
  U1-18-CDR-2l
AASSLQS

SEQ ID NO: 342 - protein, 9 aa, Artificial
  U1-18-CDR-3l
LQHNSYPWT

SEQ ID NO: 343 - protein, 12 aa, Artificial
  U1-19-CDR-1h
GGSISSGDYYWS

SEQ ID NO: 344 - protein, 16 aa, Artificial
  U1-19-CDR-2h
YIYYSGSTYYNPSLKS

SEQ ID NO: 345 - protein, 12 aa, Artificial
  U1-19-CDR-3h
GDYDFWSGEFDY

SEQ ID NO: 346 - protein, 12 aa, Artificial
  U1-20-CDR-1h
GGSISSGGYYWS

SEQ ID NO: 347 - protein, 16 aa, Artificial
  U1-20-CDR-2h
YIYDSGSTYYNPSLKS

SEQ ID NO: 348 - protein, 19 aa, Artificial
  U1-20-CDR-3h
DQGQDGYSYGYGYYYGMDV

SEQ ID NO: 349 - protein, 11 aa, Artificial
  U1-20-CDR-1l
QASQDISNYLN

SEQ ID NO: 350 - protein, 7 aa, Artificial
  U1-20-CDR-2l
VASNLET

SEQ ID NO: 351 - protein, 9 aa, Artificial
  U1-20-CDR-3l
QQCDNLPLT

SEQ ID NO: 352 - protein, 12 aa, Artificial
  U1-21-CDR-1h
GGSISSGDYYWS

SEQ ID NO: 353 - protein, 16 aa, Artificial
  U1-21-CDR-2h
YIYYSGSTYYNPSLKS

SEQ ID NO: 354 - protein, 12 aa, Artificial
  U1-21-CDR-3h
ADYDFWSGYFDY

SEQ ID NO: 355 - protein, 11 aa, Artificial
  U1-21-CDR-1l
RASQDIRNDLG

SEQ ID NO: 356 - protein, 7 aa, Artificial
  U1-21-CDR-2l
AASRLQS

SEQ ID NO: 357 - protein, 9 aa, Artificial
  U1-21-CDR-3l
LQHNSYPWT

SEQ ID NO: 358 - protein, 12 aa, Artificial
  U1-22-CDR-1h
GGSISSGDYYWS

SEQ ID NO: 359 - protein, 16 aa, Artificial
  U1-22-CDR-2h
YIYYSGSTYYNPSLKS

SEQ ID NO: 360 - protein, 12 aa, Artificial
  U1-22-CDR-3h
ADYDFWSGYFDY

SEQ ID NO: 361 - protein, 11 aa, Artificial
  U1-22-CDR-1l
RASQGIRNDLG

SEQ ID NO: 362 - protein, 7 aa, Artificial
  U1-22-CDR-2l
AASSLQN

SEQ ID NO: 363 - protein, 9 aa, Artificial
  U1-22-CDR-3l
LQHNSYPWT

SEQ ID NO: 364 - protein, 12 aa, Artificial
  U1-23-CDR-1h
GGSISSGDYYWS

SEQ ID NO: 365 - protein, 16 aa, Artificial
  U1-23-CDR-2h
YIYYSGSTYYNPSLKS

SEQ ID NO: 366 - protein, 12 aa, Artificial
  U1-23-CDR-3h
ADYDFWSGYFDY

SEQ ID NO: 367 - protein, 11 aa, Artificial
  U1-23-CDR-1l
RASQGIRNDLG

SEQ ID NO: 368 - protein, 7 aa, Artificial
  U1-23-CDR-2l
AASSLQS

SEQ ID NO: 369 - protein, 9 aa, Artificial
  U1-23-CDR-3l
LQHNSYPWT

SEQ ID NO: 370 - protein, 12 aa, Artificial
  U1-24-CDR-1h
GGSISSGDYYWS

SEQ ID NO: 371 - protein, 16 aa, Artificial
  U1-24-CDR-2h
YIYYSGSTYYNPSLKS

SEQ ID NO: 372 - protein, 12 aa, Artificial
  U1-24-CDR-3h
ADYDFWNGYFDY

SEQ ID NO: 373 - protein, 11 aa, Artificial
  U1-24-CDR-1l
RASQGIRNDLG

SEQ ID NO: 374 - protein, 7 aa, Artificial
  U1-24-CDR-2l
AASSLQS

SEQ ID NO: 375 - protein, 9 aa, Artificial
  U1-24-CDR-3l
LQHNNYPWT

SEQ ID NO: 376 - protein, 12 aa, Artificial
  U1-25-CDR-1h
GGSISSGDYYWS

SEQ ID NO: 377 - protein, 16 aa, Artificial
  U1-25-CDR-2h
YIYYSGSTYYNPSLKS

SEQ ID NO: 378 - protein, 12 aa, Artificial
  U1-25-CDR-3h
ADYDFWSGYFDY

SEQ ID NO: 379 - protein, 11 aa, Artificial
  U1-25-CDR-1l
RASQGIRNDLG

SEQ ID NO: 380 - protein, 7 aa, Artificial
  U1-25-CDR-2l
AASSLQN

SEQ ID NO: 381 - protein, 9 aa, Artificial
  U1-25-CDR-3l
LQHNSYPWT

SEQ ID NO: 382 - protein, 12 aa, Artificial
  U1-26-CDR-1h
GGSISSGDYYWS

SEQ ID NO: 383 - protein, 16 aa, Artificial
  U1-26-CDR-2h
YIYYSGSTYYNPSLKS

SEQ ID NO: 384 - protein, 12 aa, Artificial
  U1-26-CDR-3h
ADYDFWSGYFDF

SEQ ID NO: 385 - protein, 11 aa, Artificial
  U1-26-CDR-1l
RASQGIRNDLG

SEQ ID NO: 386 - protein, 7 aa, Artificial
  U1-26-CDR-2l
AASSLQS

SEQ ID NO: 387 - protein, 9 aa, Artificial
  U1-26-CDR-3l
LQHNGYPWT

SEQ ID NO: 388 - protein, 12 aa, Artificial
  U1-27-CDR-1h
GGSISSGDYYWS

SEQ ID NO: 389 - protein, 16 aa, Artificial
  U1-27-CDR-2h
YIYYSGSTYYNPSLKS

SEQ ID NO: 390 - protein, 12 aa, Artificial
  U1-27-CDR-3h
ADYDFWSGYFDF

SEQ ID NO: 391 - protein, 11 aa, Artificial
  U1-27-CDR-1l
RASQGIRNDLG

SEQ ID NO: 392 - protein, 7 aa, Artificial
  U1-27-CDR-2l
AASSLQS

SEQ ID NO: 393 - protein, 9 aa, Artificial
  U1-27-CDR-3l
LQHNGYPWT

SEQ ID NO: 394 - protein, 12 aa, Artificial
  U1-28-CDR-1h
GGSISSGDYYWS

SEQ ID NO: 395 - protein, 16 aa, Artificial
  U1-28-CDR-2h
YIYYSGSTYYNPSLKS

SEQ ID NO: 396 - protein, 12 aa, Artificial
  U1-28-CDR-1l
ADYDFWSGYFDS

SEQ ID NO: 397 - protein, 11 aa, Artificial
  U1-28-CDR-1l
RASQGIRNDLG

SEQ ID NO: 398 - protein, 7 aa, Artificial
  U1-28-CDR-2l
AASSLQS

SEQ ID NO: 399 - protein, 9 aa, Artificial
  U1-28-CDR-3l
LQHNGYPWT

SEQ ID NO: 400 - protein, 10 aa, Artificial
  U1-29-CDR-1h
GFTFNSYDMH

SEQ ID NO: 401 - protein, 17 aa, Artificial
  U1-29-CDR-2h
VIWYDGSNKYYADSVKG

SEQ ID NO: 402 - protein, 17 aa, Artificial
  U1-29-CDR-3h
DRLCTNGVCYEDYGMDV

SEQ ID NO: 403 - protein, 11 aa, Artificial
  U1-29-CDR-1l
QASQDISNYLN

SEQ ID NO: 404 - protein, 7 aa, Artificial
  U1-29-CDR-2l
DASNLET

SEQ ID NO: 405 - protein, 9 aa, Artificial
  U1-29-CDR-3l
QHYDTLPLT

SEQ ID NO: 406 - protein, 12 aa, Artificial
  U1-30-CDR-1h
GGSISSGDYYWS

SEQ ID NO: 407 - protein, 16 aa, Artificial
  U1-30-CDR-2h
YIYYSGTTYYNPSLKS

SEQ ID NO: 408 - protein, 12 aa, Artificial
  U1-30-CDR-3h
ADYDFWSGYFDY

SEQ ID NO: 409 - protein, 11 aa, Artificial
  U1-30-CDR-1l
RAGQGIRNDLG

SEQ ID NO: 410 - protein, 7 aa, Artificial
  U1-30-CDR-2l
AASSLQS

SEQ ID NO: 411 - protein, 9 aa, Artificial
  U1-30-CDR-3l
LQHNSYPWT

SEQ ID NO: 412 - protein, 10 aa, Artificial
  U1-31-CDR-1h
GYTFTNYGIS

SEQ ID NO: 413 - protein, 17 aa, Artificial
  U1-31-CDR-2h
WISAYDGYRNYAQKLQG

SEQ ID NO: 414 - protein, 13 aa, Artificial
  U1-31-CDR-3h
DVQDYGDYDYFDY

SEQ ID NO: 415 - protein, 11 aa, Artificial
  U1-31-CDR-1l
RASQSISSYLN

SEQ ID NO: 416 - protein, 7 aa, Artificial
  U1-31-CDR-2l
AASSLQS

SEQ ID NO: 417 - protein, 9 aa, Artificial
  U1-31-CDR-3l
QQSYSTPIT

SEQ ID NO: 418 - protein, 12 aa, Artificial
  U1-32-CDR-1h
GGSISSGDYYWS

SEQ ID NO: 419 - protein, 16 aa, Artificial
  U1-32-CDR-2h
YIYYSGTTYYNPSLKS

SEQ ID NO: 420 - protein, 12 aa, Artificial
  U1-32-CDR-3h
ADYDFWSGYFDY

SEQ ID NO: 421 - protein, 11 aa, Artificial
  U1-32-CDR-1l
RAGQGIRNDLG

SEQ ID NO: 422 - protein, 7 aa, Artificial
  U1-32-CDR-2l
AASSLQS

SEQ ID NO: 423 - protein, 9 aa, Artificial
  U1-32-CDR-3l
LQHNSYPWT

SEQ ID NO: 424 - protein, 12 aa, Artificial
  U1-33-CDR-1h
GGSISSGDYYWS

SEQ ID NO: 425 - protein, 16 aa, Artificial
  U1-33-CDR-2h
YIYYSGSTYYNPSLKS

SEQ ID NO: 426 - protein, 12 aa, Artificial
  U1-33-CDR-3h
ADYDFWSGHFDC

SEQ ID NO: 427 - protein, 11 aa, Artificial
  U1-33-CDR-1l
RASQGIRDDLG

SEQ ID NO: 428 - protein, 7 aa, Artificial
  U1-33-CDR-2l
AESSLQS

SEQ ID NO: 429 - protein, 9 aa, Artificial
  U1-33-CDR-3l
LQHHSYPWT

SEQ ID NO: 430 - protein, 10 aa, Artificial
  U1-34-CDR-1h
GYTFTNYGIS

SEQ ID NO: 431 - protein, 17 aa, Artificial
  U1-34-CDR-2h
WISAYDGYRNYAQKLQG

SEQ ID NO: 432 - protein, 13 aa, Artificial
  U1-34-CDR-3h
DVQDYGDYDYFDY

SEQ ID NO: 433 - protein, 11 aa, Artificial
  U1-34-CDR-1l
RASQSISSYLN

SEQ ID NO: 434 - protein, 7 aa, Artificial
  U1-34-CDR-2l
AASSLQS

SEQ ID NO: 435 - protein, 9 aa, Artificial
  U1-34-CDR-3l
QQSYSTPIT

SEQ ID NO: 436 - protein, 10 aa, Artificial
  U1-35-CDR-1h
GFTFSDYYMS

SEQ ID NO: 437 - protein, 17 aa, Artificial
  U1-35-CDR-2h
YISSSGNNIYHADSVKG

SEQ ID NO: 438 - protein, 14 aa, Artificial
  U1-35-CDR-3h
ERYSGYDDPDGFDI

SEQ ID NO: 439 - protein, 11 aa, Artificial
  U1-35-CDR-1l
QASQDISNYLS

SEQ ID NO: 440 - protein, 7 aa, Artificial
  U1-35-CDR-2l
DASNLET

SEQ ID NO: 441 - protein, 9 aa, Artificial
  U1-35-CDR-3l
QQYDNPPCS

SEQ ID NO: 442 - protein, 12 aa, Artificial
  U1-36-CDR-1h
GGSISSGYYYWS

SEQ ID NO: 443 - protein, 16 aa, Artificial
  U1-36-CDR-2h
YIYYSGTTYYNPSFKS

SEQ ID NO: 444 - protein, 12 aa, Artificial
  U1-36-CDR-3h
ADYDFWSGHFDY

SEQ ID NO: 445 - protein, 11 aa, Artificial
  U1-36-CDR-1l
RASQGIRNDLG

SEQ ID NO: 446 - protein, 7 aa, Artificial
  U1-36-CDR-2l
AASSLQS

SEQ ID NO: 447 - protein, 9 aa, Artificial
  U1-36-CDR-3l
LQHNSYPWT

SEQ ID NO: 448 - protein, 10 aa, Artificial
  U1-37-CDR-1h
GYTFTSYGIS

SEQ ID NO: 449 - protein, 17 aa, Artificial
  U1-37-CDR-2h
WISAYDGHTNYAQKLQG

SEQ ID NO: 450 - protein, 13 aa, Artificial
  U1-37-CDR-3h
DPHDYSNYEAFDF

SEQ ID NO: 451 - protein, 11 aa, Artificial
  U1-37-CDR-1l
RASQSISSYLN

SEQ ID NO: 452 - protein, 7 aa, Artificial
  U1-37-CDR-2l
AASSLQS

SEQ ID NO: 453 - protein, 9 aa, Artificial
  U1-37-CDR-3l
QQSYSTPIT

SEQ ID NO: 454 - protein, 12 aa, Artificial
  U1-38-CDR-1h
GFSLSTSGVGVG

SEQ ID NO: 455 - protein, 16 aa, Artificial
  U1-38-CDR-2h
LIYWNDDKRYSPSLKS

SEQ ID NO: 456 - protein, 9 aa, Artificial
  U1-38-CDR-3h
RDEVRGFDY

SEQ ID NO: 457 - protein, 16 aa, Artificial
  U1-38-CDR-1l
RSSQSLVYSDGYTYLH

SEQ ID NO: 458 - protein, 7 aa, Artificial
  U1-38-CDR-2l
KVSNWDS

SEQ ID NO: 459 - protein, 9 aa, Artificial
  U1-38-CDR-3l
MQGAHWPIT

SEQ ID NO: 460 - protein, 10 aa, Artificial
  U1-39-CDR-1h
GFTVSSNYMS

SEQ ID NO: 461 - protein, 16 aa, Artificial
  U1-39-CDR-2h
VIYSGGSTYYADSVKG

SEQ ID NO: 462 - protein, 6 aa, Artificial
  U1-39-CDR-3h
GQWLDV

SEQ ID NO: 463 - protein, 16 aa, Artificial
  U1-39-CDR-1l
RSSQSLLHSNGYNYLD

SEQ ID NO: 464 - protein, 7 aa, Artificial
  U1-39-CDR-2l
LGFHRAS

SEQ ID NO: 465 - protein, 9 aa, Artificial
  U1-39-CDR-3l
RQALQTPLT

SEQ ID NO: 466 - protein, 12 aa, Artificial
  U1-40-CDR-1h
GGSISSGGYYWS

SEQ ID NO: 467 - protein, 16 aa, Artificial
  U1-40-CDR-2h
YIYSSGSTYYNPSLKS

SEQ ID NO: 468 - protein, 15 aa, Artificial
  U1-40-CDR-3h
DRELELYYYYYGMDV

SEQ ID NO: 469 - protein, 16 aa, Artificial
  U1-40-CDR-1l
RSSQSLLYSNGYNYLD

SEQ ID NO: 470 - protein, 7 aa, Artificial
  U1-40-CDR-2l
LGSNRAS

SEQ ID NO: 471 - protein, 9 aa, Artificial
  U1-40-CDR-3l
MQALQTPLT

SEQ ID NO: 472 - protein, 12 aa, Artificial
  U1-41-CDR-1h
GGSISSGGYYWS

SEQ ID NO: 473 - protein, 16 aa, Artificial
  U1-41-CDR-2h
YIYYSGSTYYNPSLKS

SEQ ID NO: 474 - protein, 15 aa, Artificial
  U1-41-CDR-3h
DRELEGYSNYYGVDV

SEQ ID NO: 475 - protein, 11 aa, Artificial
  U1-41-CDR-1l
RASQAISNYLN

SEQ ID NO: 476 - protein, 7 aa, Artificial
  U1-41-CDR-2l
AASSLQS

SEQ ID NO: 477 - protein, 9 aa, Artificial
  U1-41-CDR-3l
QQNNSLPIT

SEQ ID NO: 478 - protein, 10 aa, Artificial
  U1-42-CDR-1h
GYSFTSYWIG

SEQ ID NO: 479 - protein, 17 aa, Artificial
  U1-42-CDR-2h
IIYPGDSDTRYSPSFQG

SEQ ID NO: 480 - protein, 9 aa, Artificial
  U1-42-CDR-3h
HENYGDYNY

SEQ ID NO: 481 - protein, 11 aa, Artificial
  U1-42-CDR-1l
RASQSIRSYLN

SEQ ID NO: 482 - protein, 7 aa, Artificial
  U1-42-CDR-2l
AASSLQS

SEQ ID NO: 483 - protein, 9 aa, Artificial
  U1-42-CDR-3l
QQSNGSPLT

SEQ ID NO: 484 - protein, 12 aa, Artificial
  U1-43-CDR-1h
GGSISSGGYYWS

SEQ ID NO: 485 - protein, 16 aa, Artificial
  U1-43-CDR-2h
YIYYSGSTYYNPSLRS

SEQ ID NO: 486 - protein, 17 aa, Artificial
  U1-43-CDR-3h
DREREWDDYGDPQGMDV

SEQ ID NO: 487 - protein, 11 aa, Artificial
  U1-43-CDR-1l
RASQSISSYLH

SEQ ID NO: 488 - protein, 7 aa, Artificial
  U1-43-CDR-2l
AASSLQS

SEQ ID NO: 489 - protein, 9 aa, Artificial
  U1-43-CDR-3l
QQSYSNPLT

SEQ ID NO: 490 - protein, 10 aa, Artificial
  U1-44-CDR-1h
GYSFTSYWIG

SEQ ID NO: 491 - protein, 17 aa, Artificial
  U1-44-CDR-2h
IIWPGDSDTIYSPSFQG

SEQ ID NO: 492 - protein, 9 aa, Artificial
  U1-44-CDR-3h
HENYGDYNY

SEQ ID NO: 493 - protein, 11 aa, Artificial
  U1-44-CDR-1l
RASQSIRSYLN

SEQ ID NO: 494 - protein, 7 aa, Artificial
  U1-44-CDR-2l
AASSLQS

SEQ ID NO: 495 - protein, 9 aa, Artificial
  U1-44-CDR-3l
QQSISSPLT

SEQ ID NO: 496 - protein, 10 aa, Artificial
  U1-45-CDR-1h
GYTFTSYDIN

SEQ ID NO: 497 - protein, 17 aa, Artificial
  U1-45-CDR-2h
WMNPNSGDTGYAQVFQG

SEQ ID NO: 498 - protein, 16 aa, Artificial
  U1-45-CDR-3h
FGDLPYDYSYYEWFDP

SEQ ID NO: 499 - protein, 11 aa, Artificial
  U1-45-CDR-1l
RASQSISSYLN

SEQ ID NO: 500 - protein, 7 aa, Artificial
  U1-45-CDR-2l
AASSLQS

SEQ ID NO: 501 - protein, 9 aa, Artificial
  U1-45-CDR-3l
QQSYSTPLT

SEQ ID NO: 502 - protein, 12 aa, Artificial
  U1-46-CDR-1h
GDSVSSNSAAWN

SEQ ID NO: 503 - protein, 18 aa, Artificial
  U1-46-CDR-2h
RTYYRSKWYNDYAVSVKS

SEQ ID NO: 504 - protein, 17 aa, Artificial
  U1-46-CDR-3h
DLYDFWSGYPYYYGMDV

SEQ ID NO: 505 - protein, 12 aa, Artificial
  U1-47-CDR-1h
GDSVSSNSAAWN

SEQ ID NO: 506 - protein, 18 aa, Artificial
  U1-47-CDR-2h
RTYYRSKWYNDYAVSVKS

SEQ ID NO: 507 - protein, 16 aa, Artificial
  U1-47-CDR-3h
DYYGSGSFYYYYGMDV

SEQ ID NO: 508 - protein, 11 aa, Artificial
  U1-47-CDR-1l
RASQSISSYLN

SEQ ID NO: 509 - protein, 7 aa, Artificial
  U1-47-CDR-2l
AASNLQS

SEQ ID NO: 510 - protein, 9 aa, Artificial
  U1-47-CDR-3l
QQSYSTPRT

SEQ ID NO: 511 - protein, 10 aa, Artificial
  U1-48-CDR-1h
GGSISSYYWS

SEQ ID NO: 512 - protein, 16 aa, Artificial
  U1-48-CDR-2h
HIYTSGSTNYNPSLKS

SEQ ID NO: 513 - protein, 16 aa, Artificial
  U1-48-CDR-3h
EAIFGVGPYYYYGMDV

SEQ ID NO: 514 - protein, 10 aa, Artificial
  U1-49-CDR-1h
GYTFTGYYMH

SEQ ID NO: 515 - protein, 17 aa, Artificial
  U1-49-CDR-2h
WINPNIGGTNCAQKFQG

SEQ ID NO: 516 - protein, 17 aa, Artificial
  U1-49-CDR-3h
GGRYSSSWSYYYYGMDV

SEQ ID NO: 517 - protein, 16 aa, Artificial
  U1-49-CDR-1l
KSSQSLLLSDGGTYLY

SEQ ID NO: 518 - protein, 7 aa, Artificial
  U1-49-CDR-2l
EVSNRFS

SEQ ID NO: 519 - protein, 9 aa, Artificial
  U1-49-CDR-3l
MQSMQLPIT

SEQ ID NO: 520 - protein, 12 aa, Artificial
  U1-50-CDR-1h
GGSVSSGGYYWS

SEQ ID NO: 521 - protein, 16 aa, Artificial
  U1-50-CDR-2h
YIYYSGSTNYNPSLKS

SEQ ID NO: 522 - protein, 17 aa, Artificial
  U1-50-CDR-3h
GGDSNYEDYYYYYGMDV

SEQ ID NO: 523 - protein, 11 aa, Artificial
  U1-50-CDR-1l
RASQSISIYLH

SEQ ID NO: 524 - protein, 7 aa, Artificial
  U1-50-CDR-2l
AASSLQS

SEQ ID NO: 525 - protein, 9 aa, Artificial
  U1-50-CDR-3l
QQSYTSPIT

SEQ ID NO: 526 - protein, 10 aa, Artificial
  U1-51-CDR-1h
GGSISSYYWS

SEQ ID NO: 527 - protein, 16 aa, Artificial
  U1-51-CDR-2h
YIYYSGSTNYNPSLKS

SEQ ID NO: 528 - protein, 19 aa, Artificial
  U1-51-CDR-3h
DSSYYDSSGYYLYYYAMDV

SEQ ID NO: 529 - protein, 17 aa, Artificial
  U1-51-CDR-1l
KSSQSVLYSSNNKNYLA

SEQ ID NO: 530 - protein, 7 aa, Artificial
  U1-51-CDR-2l
WASTRES

SEQ ID NO: 531 - protein, 9 aa, Artificial
  U1-51-CDR-3l
QQYYTTPLT

SEQ ID NO: 532 - protein, 12 aa, Artificial
  U1-52-CDR-1h
GGSISSGGYYWS

SEQ ID NO: 533 - protein, 16 aa, Artificial
  U1-52-CDR-2h
NIYYSGSTYYNPSLKS

SEQ ID NO: 534 - protein, 15 aa, Artificial
  U1-52-CDR-3h
GGTGTNYYYYYGMDV

SEQ ID NO: 535 - protein, 12 aa, Artificial
  U1-52-CDR-1l
RASQSVSSSYLA

SEQ ID NO: 536 - protein, 7 aa, Artificial
  U1-52-CDR-2l
GASSWAT

SEQ ID NO: 537 - protein, 9 aa, Artificial
  U1-52-CDR-3l
QQYGSSPLT

SEQ ID NO: 538 - protein, 10 aa, Artificial
  U1-53-CDR-1h
GFTFSIYSMN

SEQ ID NO: 539 - protein, 17 aa, Artificial
  U1-53-CDR-2h
YISSSSSTIYYADSVKG

SEQ ID NO: 540 - protein, 10 aa, Artificial
  U1-53-CDR-3h
DRGDFDAFDI

SEQ ID NO: 541 - protein, 11 aa, Artificial
  U1-53-CDR-1l
QASQDITNYLN

SEQ ID NO: 542 - protein, 7 aa, Artificial
  U1-53-CDR-2l
DASNLET

SEQ ID NO: 543 - protein, 9 aa, Artificial
  U1-53-CDR-3l
QQCENFPIT

SEQ ID NO: 544 - protein, 12 aa, Artificial
  U1-55.1-CDR-1h
GGSVSSGGYYWN

SEQ ID NO: 545 - protein, 16 aa, Artificial
  U1-55.1-CDR-2h
YINYSGSTNYNPSLKS

SEQ ID NO: 546 - protein, 15 aa, Artificial
  U1-55.1-CDR-3h
DRELELYYYYYGMDV

SEQ ID NO: 547 - protein, 16 aa, Artificial
  U1-55-CDR-1l
RSSQSLLYSNGYKYLD

SEQ ID NO: 548 - protein, 7 aa, Artificial
  U1-55-CDR-2l
LGSNRAS

SEQ ID NO: 549 - protein, 9 aa, Artificial
  U1-55-CDR-3l
MQALQTPIT

SEQ ID NO: 550 - protein, 16 aa, Artificial
  U1-57.1-CDR-1l
RSSQSLLYSNGYKYLD

SEQ ID NO: 551 - protein, 7 aa, Artificial
  U1-57.1-CDR-2l
LGSNRAS

SEQ ID NO: 552 - protein, 9 aa, Artificial
  U1-57.1-CDR-3l
MQALQTPIT

SEQ ID NO: 553 - protein, 12 aa, Artificial
  U1-57_CDR-1h
GGSVSSGGYYWN

SEQ ID NO: 554 - protein, 16 aa, Artificial
  U1-57_CDR-2h
YINYSGSTNYNPSLKS

SEQ ID NO: 555 - protein, 15 aa, Artificial
  U1-57_CDR-3h
DRELELYYYYYGMDV

SEQ ID NO: 556 - protein, 10 aa, Artificial
  U1-58-CDR-1h
GFTFSSYGMH

SEQ ID NO: 557 - protein, 17 aa, Artificial
  U1-58-CDR-2h
VIWYDGSNKYYADSVKG

SEQ ID NO: 558 - protein, 12 aa, Artificial
  U1-58-CDR-3h
AARLDYYYGMDV

SEQ ID NO: 559 - protein, 11 aa, Artificial
  U1-58-CDR-1l
RASQSINSYLN

SEQ ID NO: 560 - protein, 7 aa, Artificial
  U1-58-CDR-2l
GASGLQS

SEQ ID NO: 561 - protein, 9 aa, Artificial
  U1-58-CDR-3l
QQSYSSPLT

SEQ ID NO: 562 - protein, 10 aa, Artificial
  U1-59-CDR-1h
GGSFSGYYWS

SEQ ID NO: 563 - protein, 16 aa, Artificial
  U1-59-CDR-2h
EINHSGSTNYNPSLKS

SEQ ID NO: 564 - protein, 9 aa, Artificial
  U1-59-CDR-3h
DKWTWYFDL

SEQ ID NO: 565 - protein, 17 aa, Artificial
  U1-59-CDR-1l
RSSQSVLYSSSNRNYLA

SEQ ID NO: 566 - protein, 7 aa, Artificial
  U1-59-CDR-2l
WASTRES

SEQ ID NO: 567 - protein, 9 aa, Artificial
  U1-59-CDR-3l
QQYYSTPRT

SEQ ID NO: 568 - protein, 12 aa, Artificial
  U1-61.1-CDR-1h
GVSISSGGYYWS

SEQ ID NO: 569 - protein, 16 aa, Artificial
  U1-61.1-CDR-2h
YIYYSGSTYYNPSLKS

SEQ ID NO: 570 - protein, 16 aa, Artificial
  U1-61.1-CDR-3h
DSESEYSSSSNYGMDV

SEQ ID NO: 571 - protein, 11 aa, Artificial
  U1-61.1-CDR-1l
RASQTISSYLN

SEQ ID NO: 572 - protein, 7 aa, Artificial
  U1-61.1-CDR-2l
AASSLQG

SEQ ID NO: 573 - protein, 9 aa, Artificial
  U1-61.1-CDR-3l
QQSYSNPLT

SEQ ID NO: 574 - protein, 12 aa, Artificial
  U1-61-CDR-1h
GVSISSGGYYWS

SEQ ID NO: 575 - protein, 16 aa, Artificial
  U1-61-CDR-2h
YIYYSGSTYYNPSLKS

SEQ ID NO: 576 - protein, 16 aa, Artificial
  U1-61-CDR-3h
DSESEYSSSSNYGMDV

SEQ ID NO: 577 - protein, 10 aa, Artificial
  U1-62-CDR-1h
GYSFTSYWIG

SEQ ID NO: 578 - protein, 17 aa, Artificial
  U1-62-CDR-2h
IIYPGDSDTRYSPSFQG

SEQ ID NO: 579 - protein, 12 aa, Artificial
  U1-62-CDR-3h
QMAGNYYYGMDV

SEQ ID NO: 580 - protein, 12 aa, Artificial
  U1-62-CDR-1l
RASQSVISIYLA

SEQ ID NO: 581 - protein, 7 aa, Artificial
  U1-62-CDR-2l
GASSRAT

SEQ ID NO: 582 - protein, 9 aa, Artificial
  U1-62-CDR-3l
QQYGSSPCS

SEQ ID NO: 583 - protein, 447 aa, Artificial Sequence
  Antibody
QVQLQQWGAGLLKPSETLSLTCAVYGGSFSGYYWSWIRQPPGKGLEWIGEINHSGSTNYNPSLKSRVTISVETSKNQFSLKLSSVTAADTAVYYCARDKWTWYFDLWGRGTLVTVSSASTKGPSVFPLAPSSKSTSGGTAALGCLVKDYFPEPVTVSWNSGALTSGVHTFPAVLQSSGLYSLSSVVTVPSSSLGTQTYICNVNHKPSNTKVDKRVEPKSCDKTHTCPPCPAPELLGGPSVFLFPPKPKDTLMISRTPEVTCVVVDVSHEDPEVKFNWYVDGVEVHNAKTKPREEQYNSTYRVVSVLTVLHQDWLNGKEYKCKVSNKALPAPIEKTISKAKGQPREPQVYTLPPSREEMTKNQVSLTCLVKGFYPSDIAVEWESNGQPENNYKTTPPVLDSDGSFFLYSKLTVDKSRWQQGNVFSCSVMHEALHNHYTQKSLSLSPGK

SEQ ID NO: 584 - protein, 220 aa, Artificial Sequence
  Antibody
DIEMTQSPDSLAVSLGERATINCRSSQSVLYSSSNRNYLAWYQQNPGQPPKLLIYWASTRESGVPDRFSGSGSGTDFTLTISSLQAEDVAVYYCQQYYSTPRTFGQGTKVEIKRTVAAPSVFIFPPSDEQLKSGTASVVCLLNNFYPREAKVQWKVDNALQSGNSQESVTEQDSKDSTYSLSSTLTLSKADYEKHKVYACEVTHQGLSSPVTKSFNRGEC